European Patent Application EP 4 653 531 A1, published November 26, 2025. Title: Antisense Oligomers Targeting GFRAL and Use Thereof. Applicant: Korea Advanced Institute of Science and Technology. The sequence listing filed with the application follows.

SEQUENCE LISTING (37 sequences)

SEQ ID NO: 1 - DNA, 75025 bp, Homo sapiens
  source 1..75025: mol_type = genomic DNA
ttattctggacagttactcttaagaaagttgtcagaagaaacgcatctgcctttttttccaggtgaactgccgtgagttgtccagcatgatagtgtttattttcttgggtaagtgaatggtgcttctggtttatctgaattattcataatactaattctttgtaaactgaataccatcacacttaagcttaacaggggcttataatatgaagtaccaagtaaattacaaatttatgctttaacatggtttattcttcttgcaaaaatgtacactcacttttactcacttatttctaactctatagataatgcagcatgtgaaaattgtattaatctctcagcttgtttctgttttattgtatagaatgacccaatgactttgagttacttattaggattaatggaattcacacatgtgttagaaccttttagaaataaaaataaaaccttccagtatctatttacaagttataagatgaaaaatttcaaactgttatctattttatttattttgctttgaaattaaacaaaaataagattaatttaaaacattcaatttacctacagtgttaatatttgctaactagaagtaatttagtgaagtaaaaccacttaacaccatatcagaatgcttcatattttcattaatttttatgacctagaactcaagtgtggacttacttctcttgtattggatccgatgaatgtattataagatgttgatgaaaaataatttatttttatttaatgtagaatccatgaatctatttgctagatgtgtgactggagaatattttatatcttctttagcatttggtagaatctataaactgaattcagaaaaggaataattgtaactgtagctagattgtaattttaaaaatatggcattttatgtttaagctaatatatacttgaataaaggcataattatgggccagaaagcaaagaagtttactttaaattgtatcgaacataaaaggagagtcatatcaagtcaaggaaacaagttaagaaggagagaaatcccttatattttcagtttttcttttgtttaagtaatatttttccattgttccataattttgctttttgtaattattcctaaaatattttcttatttttataaagattgttaatatttctttagttcttttttgtgataaagagaaatataggaaactttaatttttatagatcaggcagcaatataatgaagctcacaaaatacattacagactcattatgacctcagttgaaaaggcaatggcctcttattttcatcttttacttctaaattaacttgacaccaggttgcatgaaggagggaaataacttcttaacattgttagaactaaaattatactatttgatatgttgtaccaacatttcccatattatattttttagaatgcttgtttgacattatctaaataggtcttataatgaggaaaatgtctgttggtaaagaaatgtggaaaacaatgaattttaaaatctcagaacatttagtaggataataagccccatacatctttaaaacactgatataatttgcagcattatccatcttattaatttaaaaatagaagttatttttcattgagtattacaggaaaattcttgaaaaatcctaggttaaatacaaaaccacaagtcatagtttggaatgaataagacagattttggagaggtaatacattcttgattcttgtggaccaaatcattgaggtggttttcttagttgagtcaatattttgttgagtaggaagtgtggaaaatcctataaaataatctattaagaagcttgttcaaccaaaaactgaaaatgtgaaaggaagtaaaacattaaaaactgaaaatgtgaaaggaagtaaaacatatttggggaagacaacatgtagtatttctaagtgattattactctgaagtactgatgaagttttgatgatatatctgggatattatcacttataagattcttgaaggggcttttcacaagatataatgattaatggcaaataaaataccattttcttataagttgagtttatgacttcaaatttctatttctgggtctttggaaaactggatttgaccaagtaaatttgtgctaggatcaaaagagtcctctttttctttctttgggctagccaaataaggagtacaagggcttggctagatgaggttgtccatgaacacatgagaaaacagaaagctgatatgtccatttccactccagccctcagcaagaaaaatgttaccaagctacacccatgggcctaatctccaaatgcagtgacccagcaagtagtacacatggtccaatcagttgtcttggattcttcttataagatgagatttgcaaagaggtaagatttaaaaaaaaaagagagatttcaagcccttacttgaagcctatcactctacattgtcacaggtgattcataattaacaacagcatttaaaaattcaaataatttggctcttatttagttatagcttgactctcttgatgacagttactacaactgtctctgtaacacaatttcaatccctgtatttttttctattaattgatttggctagtgtcacttcatatgtttgcagaatcaatttgactaacttgcgtaacatattaaattaacattgctattttcttgattgtttttagaaaacttgctggatttctcctctagcaaaagtaacttgtaaatatctggaaggtattattttttagatgttatcagttatttatatatcttatatataaacatctaataacttgggtataagccaatattcatttattgaatacctatactgcatcactgtgtttggtgacaaaaatacagttataaattatccttaatgtctgtgggtaaagctgtacaatccagtggtggagacaggcacatgaatatatacactacagaacagtaaaatctgtaattgcgggatccccacagttctagtaaatggatggaagatgtcaaattcaatttgagtgtggaaaaaggggagtatagaattcaagtaaagtttccagaaaatagctaatgattgtgttcagttttaaacaacaaaaagggttattccagaagaaaaagaaagaaaatacttatcagggatcagacagtaggtatgcagaggtagaagacagcatggatcattcgggaaacgataaatgcttgagaccttccagattgcacatggtgaggaatatgagagccctgatatgagaaatagtttaaaggatataaaacagaaaaatggcaagactagaatagtacatcaggtagattaggggttacaaagaacctatctgaataaggttctgaataagattcaaactggaggcagactgactaataagttaaacaaatgctcaaagtgaaagtcaataaatttagcaagaatgaatatgggagagtgaagttgaggatggaaaatagtctaccacaaaaccaagatttctagtttgagttctcatgttaattgtggcattgtgaatgaagtagtggtccacagtggaacaatgatgatgaagatcctgtgaaagtgtttctgaaacattcaagtagagataacaattacgtacctatgacaggaacgctggaaatactgagattaaattatacatttgagaatcatcagactaacattttagttcaaaccataagagtacatggaattttctgcagagaatgtataaaatgaaaatagaaaaggtctgagaagagaacctaagctaaaattatactttactagaagaataaaatgatcctgggaataattttagctatggtcagaaaatacaaagtggataaatatcaagagaacagaagggagggctggcaaaggaagagtttcaaaaacaaaaaagtcaacaaaatggtcaatggtgagataaagtttaaaaccattaagttagattttaaaggggtaattagagacttttttaagagcagttttaatggaataatagtaataaaaataaattataagttgaggaataaatagatgatgagacgtcaaaatgagcaaatttaaaatattcatttaagaatctataaaaagaaatacagatctacagctagagaggaggttaaggttattcccaccatcaattatttcactacatgttattttccataattctgctctttatcattaataacttagatttgaagaaaatggatgccaaatttatattacaaccttgtttttgttgttgttattcaagctatggggttaagcttggaaaatgaatacacttcccaaaccaataattgcacatatttaagagagcaatgcttacgtgatgcaaatggatgtaaacatgcttggagagtaatggaagatgcctgcaatgattcaggtaaacaagttgctaaaaatacactcaaatgatttatttttactaagataaaaacaggatttgatattttgtcattatcctaagaactaagtttttttctatgtatcttatttaatcttgacccccatcgattcacttttaatcatgtattagcaaatttaattacaaaaggattttcttaattactaaagagctttaattactgagggcagcattattcaagatttcagattattttcttacctctctcaccatgtataatgctacaattttatgcattcttctgagaaccatggcactattttttttcaaataaaaggttattttgattacatatgtcaatgataaaatagaaaaaataagatttgttataataattgttgtgcatttgtccatgcacaatgtacaatgtatattcttgaaacatatatgcggtatttccaattctatgtcaagaacaagtaaagctatagttttgtttttaacttggcctaccttccaaacatttgtggggaggttcaagagttgagaatgtgaagattggagagtgactggtattttctttcttttttctttttttttttattttgagactgaatcttggtctgtcgccaggctggagtgtagctgcgtgatctcggctcactgcaacctccgcctcccgggttcaaacgattctttctcctgcctcagcctccagagtagctgggactacaggcgcatgccaccatgcccagctaatttttgtatttttagtagagacgggatttcaccacgttggccaggatggtctcaatttcttggcctcgtgatctgcctgcctcggcctcccaaagtgctgggattgcaggcgtgcaccaccgtgcctggcctatatttccttaaaaagaaaaaatatatatattttgaatattcaagtagctaaataagcattgaatgagaacattatagtaagactcctttcattaaaagtaaatagaatagtataaactacaaatagaataaagtaaatagaataagtaaatagaataaactgtctatgtggtagaacatagtcaatttatacagtagaacattgttctacagcataatctatacagattacagtataatctatctacagtataatctaaaaataatctatttattttgatgattaaacttcttgctacattttataaggcaatttaaaatatgttgttaaaatattatatttaggtgtcacaaattgtaccttatttaatttcagtatacaaatagtcttttgcagtaaattgcaataatatttgcataattattttatgtatgaagctgaaatatgcgtattctcaaatgtacaaatgaaataaactaaggtagttttattcagaataataaataaaagaaaatgttcaggtagaggattacatatttttaaattaatgtagaaaatgaaatattggtaattatgagacttattcaataatatttattgagtgctatgtgccaggaccacataatttttaatgataaatttagagctacctgcacatatctttctatagtctgagaatgatatgaaaataaaagatcagattatgacaaaatagctaataaaatagataagctgacaaaatgctaagattagagagcattctggtcacctcctgtaagagtagccttatttttactgaaaagcaagaaatgatattctaagtaggaaaaagctattttgaaatgcagaaagttttaatatagaaagtacattatggaaaatattcaatgaaaatacaggtttttcataaaatgtcacttatatggatatcttgcagcaaccccagataatcttaccatattaattaattattcaggttaatatgttaaaagtactttggggaggaagaatccaaaattataatcagattaatatctatagtgttatgtgtttgattgtgagatccaggtgacccctgcaagatgaggaattcatcatactgtaacctgagtatccagtacttagtggaaagcaatttccaatttaaagagtgtctttgcactgatgacttctattgtactgtgaacaaactgcttggaaaaaaatgtatcaataaatcaggtaatattttgttttaagaaatgtttatagtcatgaaaaagaaagcaacaatttcaaaattaaccacatctatgtaatgtgattaatgttttttgtaatttgattaattcttttcaaagctttattattttaaaaattttgttggtatatagtaggtgtatctatttgaggggtacatgaggtgttttgatacagttcttgatgtaccttggggttctgtgagccatagacctcagtaagtgcacgacatacttctttcattactaaccacaattctaagcttcattcgagtcagtggaattatagattcactcattcaattcatatatttgtggagtttattgtggccttgcacaaaacctagatgatagaaggcaaataagatattatctttgttgttaaggaactcagtgtctcctgggagaaatcaaaatgtaactaattgctagagttatacttgcctttgcatagggacatttaatcaggctaatacactggagtaggggtgatcagttagcctgcatgtacccttaactgtacaacaaagacattccaagagatgtgcgagatcaaacagttctaaagtcaacagtttccagtcttcaatgtccctatatactccgaaaagtaatcagcagaggaatgcacctgttatcacagagtgctcaattcttctttcacaatcaaccttctctcactttacaagaggtagatttacctctcatctacacggaatggtctcatcgtccaatccaacccattcaaccatccgttgtgggctcattggacaaatttctgttccataattttgccatttccagaatatcaacaaatgaagttatgcaacatgtagccgttttaattcagtttattttgtttaacataatacattagagattcattaatttttctcatgtgtaagtttatttttcttgaagagtagtatttcattgtgtgagtatatcacaggttggttccattcattatcgaaagtaaattgcattatttccaggttttcagggattaaaaataaggctgctataaatattcacatacaagattcagacaaacataagctttacttcacttatgaaattgtggggtcacatggtaagtatatgcttaatgttacaaaaagcttctaaactgtaattcagatttagtgtaatcatcaatgtataaaagttcctgttgcttcatattcccagcaacacatttttttgccattctaatatatagtggtactatattgtagttttaatttgcacttaattataatgttaagcatatttttatatgttgtgtgccatctatctgtctatcttatttggtaaagtatttcttcaaagttttgtccattttaaaattggtgtttggttattgcattgagttttgagagctgtttctgcaagttgaatagattttttttaatcagaatatgtgttttgtatttttttagtctgtatcatttaagagtgtcttaaaaaacagaattttaaaaattttggtgaaattgagtttatcatcttttctttcatagatcatacttttgatgttgcatctaataaatatttaattcacattaacaaagattttctcataagatctagaaatgatgtagctttaggttatatatttaggcctatgttacattatgaattaatttttgtatccagtacaagatataagtcagattttcttccctgcaaatatctaattgttccacccacatttgtggaaaataatataattttacttttctcaaaagtcatttggccatatgttggtggctctatttctagactttctattctgttccattgagttaattctgtacttttgcaaatattttatagtcttactatagcttcacagaaagtcttgaaatcaagtagtatgattccattaactgttacttgaaaaataattttggctattctatttctttgtctttattttattttattttattttattttattttattttatttttgttgtgttgctgtagttgtttttgaaacagggtcttattctgccacccaggctggagcatagtggcccaatcttcactcagtgcagcctctacctcctgggttcaagtgattctcttgccaaagcctcccaagtagttgggattacaggcatgtgccaccacaccagctaagttttgtatttttagtagaaacgggttttcgccatgttggccaggctggtctgcagctcctgggctgaattgatctgcctgcctcagcttccaaaagtgctgggattacaggtgtgagccaccgggccgggccacttctttgtctttccataaacattttagaatcagcttgtcaatgtctgcaaagaatcctgctgacattttgactgaacttaccttgaaattataaaccaatttactatgtcgagtgttcagatttattaacatgatatatttcttcatttatttataacttcattgatgtagttcatcagtatttgatagttttcagtatatagttcttgcacaactttttaggcttctacaaacacacttcaggttttggtgctgttacaaatggtaatttattttacatcttaactttctattgattatagtgattatatagaaatacaattaatttttctatatggactttatagcctatgacttgctaaatgcaattattctatttttttgtagaatctgcaggaaattctaaataaatattcttgtcatctataatagagtttcattttcccctttccaatctttagtctttcatttattttccctgctttattaccccaactagagctttcaatatattaaatagaattgttgaaagtggacatcttaccttttcacctgtcttaggagaaaggcattcagttttgtaccataaagagtgtgtgtgtgtgttctttgcaggttctctttatcaagtggaggaaattccttatttttggttttcttcgtttttaaaatcataaatgtataaataaatgctgaattctgcaaatacttttttagcctctattactattaattacttcaaacatttatcttttccttttttggggagtatttctatttttctggccattttaaaatatatagtaaattagtgttaactatagtctccctactgtactatcaagtactagaacttattccttctatgttaatgtatatttgtatccgttaaccaacttctctccatttctcctcccccgtgtcctgccaagcttgatcacattttttcctttagttttttatatggcgaaattcattatttgattttttactgttgttccagcccttcatttcaaggctaaattctgttcaatcatggtgtattattctttttgtatttctggattcaactgctaatattttgtttaaaaaactatgttcataaagtatattggcatgttgatttgttttcttataatgtctttggtttggtatctaagttatgctggcctgtaaaatcaactgggaagtatttcctcctcttcaatattctggaaaagcacaaaaagaattggtgtcattccttccttacatgatctatttcattaaccagtaaagatatctggcccatgcttcattaaaaagatttgaaaatataaattcaatgtgttaacttgttgtaagactattcttgttatctatttcttcatgagtgagctttggtaatttgtgtcttccatttgctgaatttatgttggatttttatccttaaagttttcagtttactgtttctttttggtttctatctccctacaaaattgctcctagtatttcctaattgtcctttttaatatctgtagcagttgcagtgatgtcctttttatgtttacatattgataatttgtataatttgtgtcctttcaattttactattcattgtttctttatgtgtatgtctgatttgattttaatgtgttctccattttcttgcttcctaacataaaaccttgagccactgatttgagattttattctttcctcatataagcatttaatactatgaatttccttccaagtactgatttagctatagccacacattctgatatgtagttttaatttaaatttatgtcaaaatattttctccttttctttgtgacttccactttgttatgatttattttattattattattatattttgaggcagagtctctctctgtcgcccaggctggagtgcagtggagtgatctcagctcactgcaaactccttctcctgggttcaagctattcctctgcctcagcccctgagtagctgggattacaggtgcttgccaccacacctggctgatttttgtatttttagtagagacatggttttgccatgttgtccaggctggtcttgagctcctgacctcaggtgatctgccagcatcaaacttccaaagtgctgggataacaggcatgagccaccatgccgagccagaaggttatttaatttcctaatatctgagatttctcagatatcttcattattgatttctagtttaatttcagtatcataatataacatattttggatgatctcaattctcaattcttaattaaaataataattgccaaatatcacctatacaatgtgatacagtctacacacataataaggacacacacatacacacacagacaaagtactagaagccatagagtaaaaaataatggtgactcagaagacttcacagaattgttagacttgggccttttagggtaagttggtttcattaggtaggcaaaacaaaatggataatttaagcagaagaaacagaatgaagtggggagcatttggggagcaacaattcccttgttaagctggatactagaatggaaaagtatttaacactggaaagaaatcagctatttatgaaaaggaggaaggctgaacttacatatctttctaaagagattagactttaaaccgttgctatgaggagctattacatattttaaatagaggaatgtatcatcagtttctcaaaagttatcacaggcaataacgtagagaggatggaatgggaggcaaagaaagatgcaggtcaagaatatcagttaaaaagccatcaaaataatttaagagagaggtaatgcatgcctgaactaaggcaccggtcctgagaattataataaaatatatacttaaggtatatttatgaataataatcaataggaattggtgaccagttggatatgaggaatttaaaatgtattaagcgtaatctccaggtggctggcttgggacaaggggattgctatacattgagccaagaaatgaaaaattgtacaggactggggacgaaagtgatgagttgtattctgaaaacatttcatctgaggcatgctttggaatattcgagttaggaatgttggtattttttttctaaatttgcaatgataaaaaaatagtctaaaaatgtaaaggagcatgcctcatcaagctggcattgggaagcagggatcttgaggagagaaatctaaaacagagatatagaggtttatgagtagataaaaaacataaaggagagtaagactgcctgggaaaaacacaaagggaggagaaagatattttcagaagaattttatgacctatttgaagaaaccaaaaagaagttttttaaataggaaaagaaactacagagagtggaatttttgaagccaatgaaagagaggacatgaagaaaattgtcaaaattctgaaaagtcaaaaaagatagggactgataatggcattaatttgctacttagtagatattactagttttagattaattaggctgaaatgttagcatgctgaaatgcttattaaaatatttagtgagttttttcaagatggtaagacatctgaacttaatagcctaaattgccacttttagcatatcaaattttgacaaaatattgtatatcaacagaactatacatatttagagcagttaagttgaaatcagtttacatactaaaactattttttccacaatagaaatttattaaatgctgttatgtggaaatattgatgaatcaggcatacaaaaaccttgcactcgatgagagtttcatatggacaagacctaaaggagaaagcctaaatattcccgatggacttcgtaaaggacctgacctggattttgtgtttacagaaagcattcagctgatttattataattcatgacaaagaattataaagaaattgataatttaaatatgagaaagaacatgataatttaaatcttaccattccttctatgtcaactgcagcatcctccacagaccttctaatcatcacttcaacaaaatggttttctctccatgctttgcattcccaaaatattctccagagtacacagacatgcacttttctattctcaagaaaatcagttttgttatttcttttaaaaaatatgctaaagcacccagcagaatacctgacgcttagcaaattattagtaaatatataacgtaaatatttttcattaactaaatattgagcatctccatgatgtatccattaataaaatatttatgtgtaaaccctggagaatataaagagcatcatcaaatgaaatgagcaaacaaaagtggttggcagcagttccaagatggcagaataggaacagctccagtctacagctcccagcctgagtgatgcagaagacgagtgatttccacatttccaactgaggtaccaggttcatctcactggggcttgtcagacagtgggggcaggatagtgggtgcagcctactgagcgtgagctgaagcagggtgaggcattgcctcacccgggaagcacaaggggtcagggaattccctttactagccaagggaagtggtgacggatggcacctggaaaatcgggtcactctcaccctaatactgcacttttccagtggtcttagcaaatggcacaccaggagattatatcccgtgcctggcttggagggtcccacgcccatggagcctcgctcattcctagcgcagcagtctgagatcaaactgcaaggcagcagcgaggctgagggagggacgcctgtcattgctgaggcttgagaaggtagacaaagcagctgggaaactcaaactgggtggagcccatcgcagctcaaggaggcctgcttgcatctgtagactccacctctgtgggcagggcatagccgaacaaaagacagcagaaacctctgcagacttaaatgtccctgtttgacagttttgaagagaatagtggttctcgcagcacagagtttgaaatctaagaatgaacatactgccttctcaagtgggtccctgacccccaagtagcctaactgggaggcaccctccagtaggggcagactgacacctcacacagctgggtacccctgtgagacgaagcttccagaggaacgatcagacaacaacatttgctgttcagcaatatttgctgttctgcaacctctgcttctgacacccagtcaaacagggtctggagtggacctccagcaaagtccaacagacctgcagctgagggtcctgactgttagaaggaaaactaacaaacagaaaggacatccacaccaaaaccccatctatacatcaccatcatgaaagaccaaaggtagataaaaccacaaagatggggaaaaaacagagcagaaaagctgagaattctaaaaatcagagcaactctccccctccaaaggaatgcaacacctcgccagcaatggaacaaagctggatggagaatgactttgacgagttcagagaataaggtttcagatgatcaaacttctctgagctaaaggaggatgttcgaacccattgaaaagaagctaaaaaccttgaaaaaagattagacaattggttaactagaataaacagtatagagaagtccttaaatgagctgatggagctgaaaaccatggcacgagaactacatgatgaatgcacaagcttcagtagccgattcgatcaactggaagaaagagtatcagtgattgaagattaaacaaatgaaaggaagcgagaagagaagtttagagaaaaaaagagtaaaaagaaatgaacaaagcctccaagaaatatgggactatatgaaaagaccaaatctacatctgattggtgtacctgaaagtgatggggaaaatggaaccaagttggaaaacactctgcaggatactatccaggagaacttccccaatctagcaaggcagaccaacattcaaattcaggaaatacagagaatgccacaaagatattccttgagaagagcaactccaagacacataattgtcagattcaccaaagttgaaatgaaggaaaaaatgttaagggcagccagagagaaaggttgggttacccacaaagggaggcccagcagactaacagcagatctctcggcagaaactctacaagccagaagagagtggggaccaatattcaacattcttaaagaaaagaattttcaaaccagaatttcatatccagccaaactaagcttcataagtgaaggagaaataaaatactttacagaaaagcaaatgctgagagattttgtcaccactaggcctgccctaaaagagctcctgaaggaagcactaaacatggaaagggacaaccggtacccagccactgaaaaactcatgccaaattgtaaagaccatcgatgttaggaagaaactgcatcaaccaacgagcaaaataaccagctaacatcataatgacaggatcaaattcacacataacaatattaaccttaaatgtaaatgggctaaatgctccaattaaaagacacagactggcaaattggataaagagtcaagacccatcagtgtgctgtattcaggagacccatctcacgtgcagagacacacataggctcaaaataaaaggatggaggaagatctaccaagcaaatggaaaacaaaaaaaggcaggggttgcaatcctagtctctgataaaacagactttaaaacaacaaagatcaaaagagagaaagaaggccattacataatggtaaagggatcaattgaacaagaagagctaactatcctaaatatatatgcacccaatacaggagcacccagattcataaagcaagtcactagagacctacaaagagacttagactcccactcaataataatgggagattttaacaccccactgtcaacattagacagatcaatgagacaggaaggtaacaaggatatccaggaattgaactcagctctgcaccaagcagacctaatagacatctacagaactctccacccgaaatcaacagaatatacattcttctcagcaccatatcacacttattcgaaaattgaccacatagttggaagtaaagcactccttggcaaacgtaaaagaacacaaattataacaaactgtctctcagaccacggtgcaatcaaactagaactcaggattaagaaactcactccaaaccgctcaattacatggaaactgaacaacctgctcgtgaatgactgctgggtacataattaaatgaaggcagaaataaagatgttctttgaaaacaatgagaacaaagtcacaacataccagaatctctaggacacatttaaagcagtgtgtagagggaaatttatagcactaaatgcccacaaaagaaagcaggaaagatctaaaattgacaccctaacatcacaattaaaagaactagagaagcaagagcaaacacattcaaaagctagcagaaggcaagaaataactaaaatcagagcagaactgaaggaaatagagacacaaaaaacccttcaaaaaatcaatgaatccagtaactggttttttgaaaagatcaacaaaattgacagactgctaacaagactaataaagaagaaaaaagagaagaatcaaatagaagcaataaaaaatgataaaggggatatcaccatttaatacagaaatacatcccacagaaatacaagctaccatcagagaataaacacctctacacaaataaaccagaaaatcaacaagaaatggataaattcctggatgcatacactctaccaagactaaaccaggaaaaagttgaatccctgcatagaccaataacaagctctgaaattaaggcagtaattaatagcctaccaaccaaaaaaaaagtccaggaccagatggattcacagttgaattctagcagaaatacaaacaggagctggtaccattccttctgaaactattccaatcaatagaaaaagagggaatgctccctaactcattttatgagaccagcatcaacctgataacaaagcctggcaaagacacaacaaaaaaagagaattttagaccaatatccctgatgaacattgatgcaaaaatcctcaataaaatactggcaaaccgaatccagcagcacatcaaaaagcttatccaccatgatcaagtgggcttcatccctgggattcaaggctggttcaaagcatacgcaaatcaataaacataacccagcatataaacagaaccaaagacaaaaaccacatgatcatctcaatagatgcagaaaaggcctttgacaagattaaacaacgcttcatgctaaaaactctcaataaattaggtattgatgggatgtatctcaaaataataagagctatttatgacaaacccacagtcaatatcatactggatgggcaaaaactggaagcattccctttgaaaactggcacaagacagggatgccctctctcaccactcctattcaacatagtgttggaagttctggccagcgcaatcaggcaggagaaagaaataaagggtattcaattaggaaaagagaaagtcaaattgtccctgtttgcagatgacatgactgtatatttagaaaatcccatcatctcagcccaaaatctccttaagctgataagcaacttcagcaaagtctcaggatacaaaatcaatgtgcaaaaatcacaagcattcctatacaccaataatagacaaacagagagccaaatcatgagtgaactcccattcacaattgtttcaaagagaataaaatacttaggaatccaacttacaagggatgtgaaggacctcttcaaggaggactacaaaccactgctgaacagaataaaagaggacacaaacaaatcgaagagcattccatgttcatggataggaagaaccaatatcatgaaaatggccatactgcccaaggtaatttatagattcaatgccatccccatcaagctaccaatgacttccttcacagaattggaaaaaactactttaaaaagttcatatggaaccaaaaaagggcccgcattgccaagacaatcctaagccaaaagaacaaagctggaggcatcttgctacctgacttcaaactatactacaaggcagtagtaaccaaaacagcatggtactggtaccaaaacagagatatagactaatggaacagaacagagccctcagaaataataccacacatctacaaccatctgatctttgacaaacctgacaaaaacatgaaatcgggaaaggattccctgttgaataactggtgctgggaaaactggctagccatatgtggaaagctgaaactggattccttccttacaccttatacaaaaattaactcaagatggattaaagacttacatgttagacctacaaccataaaaaccctagaagaaaacctaggcaataccattcaggagataggcacgggcaaggacttcatgtctaaaataccaaaaacaatggcaacaaaagccaaaattgacaaatgggatctaattaaactaaagagcttctgtacagcaaaagaaactaccatcagagtgaacaggcaacctacagaatgggagaaaatttttgcaatctacccatctgacaaaggggtactacccagaatctacaaagaactcaaacaaatttacaagaaaaaaacaaccccatcaaaaagtgagtgaaggatatgaacagacacttctcaaaagaagacatttatgcagccaactgacacatgaaaaaatgctcactatcactggccatcagagaaatgcaaatcaaaaccacaatgagataccatctcacaccagttagaatggcgatcattaaaaaatcaggaaacaacaggtgctggagaggatgtggagaaataggaacacttttacactgttggtgggactgtaaactagttcagccattgtggaagacagtgtggcgattcctcagggatctagaactagaaataccatttgacccaaccatcccattaccaggtatatacccaaaggattacaaatcatgctgctataaagacacatgcacacgtatgtttactgcaacactattcacaatagcaaagacttggaaccaacccaaatgtccatcaatgatagacttgattaaggaaatgtggcacatatacaccatgaaatactatgcagccataaaaaaggatgagttcatgtcctttgtagggacatggatgaagctggaaaccatcattctcagcaaactatcccaaagacaaaaaaaccaaacaccgcatattgtcactcataggtgggaattgaacaatgagaacacttggacacagggaggggaacatcacacaccggggcctgtcgtggggtggtaggaggggggagggatagcattaggagatatacctaatgtaaatgatgagttaatggatgcagcacaccaacatggcgcatgtatacatatgtaaccaacctgcacgttgtgcacatgtaccctagaacttaaagtataaaagtaaaagaaaaaaaaagttgaccatatgttgagtcaaagcaaatatcaacaaatttcaagacactgaaataattagaaacatgtaattttatcttggtggaaataacctagatatcagtacaaaaaataaacaagaaatcccccccccccaaaaaaaagaaaaaacaaagtaagtgatgaagaaaaatatcaccaaaagaaattgaacattaacattatgtggttctataacctgtaatattggtggtaattaattttttaatttgttgggatgctagttaagttgatagtgtgacttttctgtgagaaaacaaaacagtataaatgagcagataaaccactcagtaaaattttatagggttggagttttatagagaatcacgggaaagtaaaagaagaaaggacgaaaagacaataacaagaaactgttcctttatctgaatgggtgagtgatataggctggaaagagtctatgaatccaggagatgatgctaagattgggagtgaataaaaagatgaaagttctggaggtatatgtgcacatgaaataatcaagaatgtgaagctttggaagcgagtaagataagtaatatttgcaattgaaagagagagaacttcatgtcaatgtcaggtctagaagtcgatcattggtgtggcatagttggagtgtcggtgaaggtcataagagctatggttaaggaattctgaattaagggtggaagatggttttgtcccaaaagacatagagataacttagcacaatgacaagatctgaggtagaggagaatattgagacagtacctgagtcgatgctgaatatcagggcaagactttgaggttaatatttgacaaaagaaaagagggaggcacaacccgacagcataaaattcaaagaaggagaaatgttttataaggatgaataattaatattttggaagctacaaagctggaaaagtagatataaacacattctaatgatatcgtggtatgatctatatgggaaatgggtaggattcactagcaagagctacagggaagtgaggctagagaaaatctaggcttcccagatattacacttttctatttttcttcttgcttccatgggtgattcttctcagtctcttttgagcatcttcttttgcttttgctttaaatgttgccacataccctctaaaaaagaaatctctgttgcatttaattcaactagtcattttatagaaacatgtttgtctactagtttattgtaagcatatttcttatcagattataaaatataaatcaaaatatttacatatacaagagtttagtttctgatattatcaatgttaagaaaaagaagatgtatggaagtacttctgattctaatattagatattagagcatattttagggattgttggatattttctgatgaactgtataggattttataactcacatgtaggtcttattggtgaatacttttatttgtttcctgaacatattgaccttcagctcctctttcagtaaaagccactgtttaaaatatcctctgggaaaaaatgagtgtgtgtgtgtgtgtgtgtgtatgtgtaaatgctagttttatatttaatgtgtaaatgttaatttcatacaaaattagcatttaatgtataagtattaaaatgtaataccttctatgaagcactttattttcagacactaaaaataactgttttgttgtgttggtaacaagtactcatatagtaagtaaattaggctgctctggctaccataacgaaatactacgggctgggtggcttaaaaagcaaaaattgtatttttccccagttccggattacgaaaaatctcagataaaggtccccagaatcttttcctggctaggactcttcttttactagcttgtagatagccagccacattttccctgcgttctcaggacctttcttcagtgagtactccaggggagagagacagctagctccctgaagtcttctgacatggacactaatcctattcgatcagggccccactcttatgacctcttttaacctaaagacaccatcaccccataactgcacacggagattatggctccaacttatgaatgtaggggtaatgagaaaaacattcagtcaataacagtgagtgaagctgttgtttatttaggtctacacagtagtttcttgaatatattttagtcagtggcacagccttaccaatcattcccaatgcaggggtactaatccataaaagaatgtccagcctagacttttgtacctgttacaaaagctatatgactccctgggatctgtttgttgggattttattagatatggaatagtagcacagaagttggaacctccagatcttcctcagagaggcgggatgatgggtgggatcaagaagaaagagtggttctcaagctgagacttgatcaattaaaaaaatgaaaaacaatgcataatgagaatagcttggacaatataaggagtctggaaggccatgacacacctgggggtagaagtaagtttcctgtgatagtaccatcttatatgtgcactagactagcaggcaggaaatatgaacaaacagctcagattaggacataatcatgaagggacatttatgccataacaaaacttattatcttaatatccaatgaaaaaataataattttcatttcaaaatgaaaatcttatcatctgattcccctgccactttatggatacattagtgctccttatagtttcttttggctttgttttatatgtctgtatttccttctgggctgtgggatgctcgatgacagggactgcagatttgcatcctcagtttgtcacctggtacatagtagggaaccaaccaatgttcctttaaagattttggaattagatgaacaccgagttcattttcgttgatgagatttttcaatactataattataatttctaagaactcttggaggataagataatcagaggtgaaactggttttaaaaattgcatttcatactaaagaagacccttctgagaagggtttttatgctgggcagggtgggaggtagtgttcagaaaatattccttctgttttttttttttttttccccagtcagcatccaatgtttgtttactccgtgcacacagtctaatcactagcatttatttaagtcttcaagtaactgaatcctcagagcagggctgtatagctcacttgaatgatatttcagaggcttgttttcttcatctataccacattaattttgaatatcaagggctaaatacatgttacataaccttgtatgtacttttgcttgaatatatgtggactttactcatttataaatgtggcccacgttttcctaggaaattcagaaaattgttcaataatgaaataatttctttgttttccttctagataacgtgaaagaggataaattcaaatggaatctaactacacgttcccatcatggtaatgtttttaagttattattttgatctgcattgcaaatacctgataatataaaatgcagttaccaggcttcttaaagataggccaatacagaacaaatcatgtggtttaacagttctaatataataaaatgcagcaaaatcatttcatttcttttactaatgatgcatcaaagcaactactttgcccatccattatcaatttatacatgcgctaagaaatacttaataattaaaaccaaatactaggttgggcacagtggctcacagctgtagtcccagtactgtgggaggctgaggtaggtggatcatttgatcccaggagtttgagaccaacctggacaacatggcaaaaccctgtctctacaaaaacaaaacaaaacaaaaacaaaaacaaaagtcaaaacttagcgggtcatgtaggcttgtgtctgtgatcccagctcattgggaggctgaggcaggaggatcacttgagcccaggagttggaggttgcagtgagctgggatcatgccactatacaacaagaccctgtctcaaaaatcaaacaaacaaaaatccaaatagtagatagtgattacatttaataggtatttgtgatcatataagttatttggcaccaactgtttttgtgtatacttgtgtatctgtaggagtataaacatttatatatgctagaataaatatgtggagcctttattcaagattcccctcacaaaaatgtgcaacagaacaagaatcattttgccttgagccaatgagctaaccataagctacatagttcaaatgcaatttctgaagatttatcgtttacatttgaaaaccttggactgggagatttttccttcagctcaattttggcccagcacgcttcccatcactctagatcacaatgtgtatcctgtatagatgaaagatgattccaataagtctacgatttaggtctcagtaaattcatacttactctaaaagatgtaatgtttgccaaaaataggacattggtacatcattgtattttgctcatagacttctcacagtgttttatagtttctgtatgtacagctttgtgtttacttttccacgacctgggcatatcattgctttcaggattcaaagggatgtggtcctgtttggaagtggcagaggcatgtgtaggggatgtggtctgtaatgcacagttggcctcttaccttaaagcttgctcagcaaatggaaatccgtgtgatctgaaacagtgccaagcagccatacggttcttctatcaaaatataccttttaacattgcccagatgttggctttttgtgactgtgctcaatctgatataccttgtcagcagtccaaagaagctcttcacagcaagacatgtgcagtgaacatggttccaccccctacttgcctcagtgtaattcgcagctgccaaaatgatgaattatgcaggtgggtaaaaacactcataccttactttcttatttcggcaccttatttgttatagtccagtcctaacacttgatctcataacattagctagagttcccaccatcatccaacatagtgtaaataaaaccagacaattaatatttttttgaatctgtggtacatatgcagtatcatctgaaattcaaatgcagagtagatttttgaaataaaaaatcagcatgtcaaaatatggtagccatgaaataatattataaaaattatgtattcaagttagactaatgaattggttaatagacctgacttacatatcagctttttaattttttttttgttgtttgtttaattatgtaaggctgttacaaatttattattttggcaaggagactcttcaaactttgaaataaattctttctgtcttaggctggagatcaggaggaagaaggtagcataaatactcacatgagtggtgcaaagtcagagataaccaggtccacacacatttgtgtcttttcacaatgtcaggctttaatactgttcaatcacaaaagccacaagctacatggagttcccaaggaggcagttctccttagtacttctcattcactttgttttcagagccatgggtacacaggctcaagccactccacaaatcagtcaatattgcaaaccatacataataatatacttaatatataaggattataggttaaacattccacaacaaagtaacatttaacattaagagaaaagggatagagaaaagggttaatgaaaaagtccaggaagagtgacaaaaacaaagattcttctggtcttatctgggctgtccattgatcttgcaaggaagagtctgatgtggggagaattgttggcagcagatgctgggtgcttatgagcgacagcaagatggtgtcaggtaagatggccattttgagctgctgaagtcctactctctttatggccacagagtcctcttgagaggaccgatagtggaagagtatgcttgtttatgtccttatttggttggatgcagtattgtttatttagcaaaatattttgtccctgttggaaaagtaccgtatgaaatctaagatggagtcttttttggagttacttatgtcaaggatgctctatacaagtaggatttggacatccctagcacacatgtatgctatgaccatagaaatgtattcattctcctctttctaacctcacacctttaattattgggggagtaatgttagtcgtttatttattaattcaaaaaaaatttatcaagcacctactactactctaggcaatggcgaataaggaaaacaaatgcctatggatcttatagtccagagagaagacagatattaaattaaaaatgtatgtgttgttttaaggcaaacaacactaggcaaacagtagatactgagagaggagatattaagcaaactgaccagccagtgcttaggaaaacatgtatgtggcattttagaaaagcagtgagggtagagtgtgcaaaggggagagaaataggagcgagataagagagttaattgagtgggtgtgaacaggcctatatcatatgagggcttgaaggacactgcctagggcttcggacatgtaggtggcttagtgtgtgatttgtcatatttgtccccttgtttcaactactggcaaaaaaacacaaaaagtaatgatatcaacttcctgaaggttcttagtaaaattctctcttttagctttttaactatgtctactcttattttcagtcactctaactggcaaagtagttccagatcttgtaaacatttgttaaaaagaactgcttccctatagcacacattctatgaaataagtggtaaagagctaagcagagtcctagagcattgacatatttcgtcaacttataggatatcaaggttcttaaaattgtattcaagaatttttcatgcaaatgtgtcagttattttaaggcttattatttatttttcttgagtgaataaggcattgacaaaatactttttataatgcaatttaggtttttcaaactcatttatcatctcaaaaatccttattagagaaatactacatttcattgattctaagatgcaatttctttttacacattttaacatctctgacatattttaaataaatttttaaggtcaataacaaagacatttgtcataatttaagttccagcaggtgttttttgttgttattgttgttgtacataaaataatggtatcttctgaaatcaatgaaatatgaaatcaatgaaatatcaaacacatgtgattacactacttttctcacctcaaatgaactaaaactattactattctgcctttctaactatcatattcctacatcaacaatgaaacctaataatattttaaccagccagggccaggggcaccatggtttcaatagcaaaatcactataaaaatatcagatttattcacagatgggtacccagctttgcctgattccagtgccagggctttcgatatgctatctaattatctggaagccattagcattcaaccttcaaagcatggtatttctgagcatccacatcaaagaaaatattttaatagcaagtggtggctctgctgctatagtccttgagaattcctgtgatagactctgaagcacacactcttacactaacctccccttggtatcaacaccttctcagatggactggcacagagttgatgattttcctcaacaaggacccccagctttaaccaccttttcaaaatgtttggtgtggggtctggagtgggataagcactcaaaaaacgtcatctcccttcctctcacttttgaatattgtacacttaattgttatattttagtatacatatatgtatttcttctcatgtaatttatttcttagattagttcaagtgtaaggactgtgtgtcttcaatttcctttcactatgtgcaaatagtcccttaatcagtactttatagaggtgatggaaatgttatataatattagtagtcaatgtgaaaagacaaatcctatcattttcctgagcacattttgccttagggagatttccagcttttatattaaattattgttaatgtaattcagatgaaaaacaaatctccaaatggaaaaccacttcttcaatgagaatattaagccctttatgatacttatcttttttgcagaagagcctgtacataggcaaaacagggcacttcagttttaaaatacaatttctgtccctgttccaaatttttcaattcacgatgggctttgaaattcctttattttttaactgccaaagagaacaatttaagggccatttctcaattacctttctctagtaccgacaccctcagggaggtgagattatgtcttgccaatttcacaaaagtctgggtatttacagaaaattataatacattatatttttatatattaacttaaaaaagtaatgacaaggtatttgcttaggaaatattctaaatacttttaaatatgtatgcattatttaattgatttaaaacagatgacatcatattatatacttctctatatattgtttttgttttttttccctaaatgtggattaaagatctttccataattgcatataagaaaattcacacatcagggtctgttagggagtcgggggcgaggggagggaacttagaggacaggtcaataggtgcagcaaacaaccatggctcatgcgtacctatgtaataaacctgcacgttctgcacatctatctcatttttcttagaataaattaaaaaaaagaaaattctcaaatgtttgaatggctatagagtatgccattgcatggatgtagcttaattaatttgcttagtcttttttggacatttagacatattccaagtatcttattttatttgtagctattgtaaatgggactactttgaagatttgtttttcagattgcttgctgttagcatatagaaatgctactgatttttgtatgttaattttatatcttgcaactttactgaatttgttgatcagttctaagagttccttggtggagtctttgggtcttttcaaatataaaattatataatctgcaaacaaatttttctacctttctaatttggatgccccccttttcttttccttctcttgtctaattgctgggctaggacttccagcactatgttgaataatagtgatgaaagtaggcatccttgtctcattacagatcatagaggaaaagctttcagtttttccccattttatatgatactagctattggtctgctctgtcatatatggcatttattctgttgaggtatattccttctatatcctggttttgaggcttttatcatgaaggaacgtagagaactttagcaaatgctttttcagcatcaattgaaaagatcatgttttatgtccttcattttgttgatatgatgtatcaaactgattgattttcatatattgaaccatccttgtatcactaggataaatcccacgtggtcatgatgaaaaatcttaatgtgttgttgcatttggtttgctaggattttgttgaggatttttgcattaatgttcttcaggaaaattgtcctgtagtttactttccttggtatgtcttgtctggttttggtattagggtgatactggcctcaaagaatgagtttggaagtattccctcctctattgttggaaatatttttagtagaattggtattagttcctctctaagtgtttggtaaaattcagcatcatgtcccaggttttcccttgctgggagactttctattatagcttcgatctcattacttgttattggtctgttcaggatttggacttctttatagttcaatcttggtaggttgtgtctacaaatttattcacttatccattttagattttctgatgtattggcatatatttgctcatagtaggcttcaatgatccttcgaatttctgtggcatcatttgtaatatttcctttttaatctctgatttcatttattgaggtcttctgtttctttttattagcctagctgatggtttggagattttatctttccaaaagaccaacttttcattttgttaatcttttgaattttttttgtttcactttcatttatttctgctctgaagtttattttctactattaattttgggttcagtttgctcttgcttttctagttctttaagatgcgttgctaagttgtttatttgaagtttttctacttttttgatgtaggtgcttatttctataaacttttctcttaatactgctttttccatatcccacaggttttggtatgttgttcttccattttcattgttttaatacacctctaaattttactcttaatttctttatttgcacactggacaatcaggagcatattgtttaatttccatgtatttgtatagttttcaaagttcctcttgtcattgatttctagttttattccattgtcatcagagaaaatacttgatatgatttcaagtttttgaaaattttaagacttgctttttagctaacatatgggttaccattgacaacgatctgcgtgctgaggagaataatgtgtattcttcagctattgtatgaaatgtcctgtaaatatctattaggtacattttatctatagtgcagattaagactgatgtttctttgttgattttctgtctgaatgatctgtccaatgctgaaagtgagatgttgaagtctctctctttaggtctaatactatttgctttacatgtctaggtactgcagtgttgggtgcatatatatttacaattgttatatcttcttgctgagttgaatctgttatcattatataatcaccttctttatctttttatagtttttttcttgaaatctattttgtctaattaaagtatagctactcctgcttctttttttggttccattggcatagaatatctttttccatccctttatttttcaatctatgtgtttctttatagatgatgtatgcttcttagaggtaacagatcattggctcgttttatttttaatccgtttaatccattcagccatactatgtcttttaattggagactttagtccatttacatttcaaataattttggaatccagtgtaccaaagtagtattttatttttaattaaatattctttagttcatcattttggcaaaatttcatggtgtttttcctgagtgaaaatttatctacttatgtataagtagataaaccatgcaatttaaacttagtaaaacatatttaaaatgaataaatagcatgtaggtacagatgtagtctctatctgaatgacaatcaatacttccaaaacttacatttagaagatatcttatatgtaacccttaacagcattgaaggaatatgtttgttcttctgacctaataattacatgttcagaaaatttgcagtatttcctttattataaatttaatatacatgaattaatcttcattattatatttaaaagcttatcctttaagatgagttaaatatttaattattaaaaacaatgtgactttggttttttaacatagcagcatccatgtggacaaataacttcatgaaaatgtcatgtacttatagggctttcatacatgtttgatgtcaacctattcaagaagagtaaaaagcaattttcggtgacaaacattaaattgaaataattttattcttgcattcattaataaaaatatattcttattgtaaaaaaattcaaaaatgaaattagtgtacattatccagactttttttcaattttattacagcaataatcaaatacatacagaaattttatacctcacaacatattgtaaattctaattagtctgtttagtctcttgagaaagtataaagcgcctcccatcctgtgggataactgacttgaaaagtcaaataccttacttgaaatcacttggtgtgacacagtggccaaaggctagccacaaaactatatttggaataaaaaattgccaataaatctctgaagcagttcatgcctcaaatagtcatacattggaataaaattagtaataaaggaaaatccatccgtggaatcctcaacttaactgctgtctttcatcacaaaaaagggacaataattcacaatattactctacaatttcttccacactacctatggtgatttttcaaatcacaaatttacttttcaactatgtactggcatctcgaaggcattgtgttctatgtctttcattaggtgaggggggatcacatgttaatgtgaaataacactattcaaaactaattatttttcttcactctttctctaggaggcactatagaacatttcagtcaaaatgctggcagcgtgtgactagaaagtgccatgaagatgagaattgcattagcaccttaagcaaacaggacctcacttgttcaggaagtgatgactgcaaagctgcttacatagatatccttgggacggtccttcaagtgcaatgtacctgtaggaccattacacaaagtgaggaatctttgtgtaagattttccagcacatgcttcatagaaaatcatgtttcagtaagttccccaaataaaattatctgtctatctatctatctatctatcatctatctatctatctattttgtttttgcctatacagtaaaagaggtaatccagcacagacatttttgtgtttggtattgcatttgaaaatttgctttctgattatgttctgtgtatttgctattttactcacttacttgaaaatagtacattttaaaaatttatatgataggtcactcttaattatcatttattgatttcaatatcaaaagcatagaaggtttattctatcagataaatggatatatcaagtatcaattgctgcataacaaaccataagtatctatactaagtaacaaaacaatggcttaaaacgataaccatttatttgctcacaattctgcacattggacttggctcagctggatggctcttccgatggtcttttggggggtcactcatgtgcctatagtcatctggtatctttaggctcggctgaggctgtttggtccaaggtggtattagcagacaccattttctggtgtggtgtggttcacttcaatatgacatcttcagcaatatagccaaaaactcttatgtggaagcagaagagttcctaatggctaaaccccattgtgtagctgtctagtatctgctactgtcacatttgtaattatttcactgaacaaagcaaatcacaatggccaacctcagagtcactgtgggagtggactacataaggatatgaatattcaaggtcagattaatcaaggatcattactctaacaacctactatgattggctgtcctggcctatgtacaatatattcactcttcaatttagtttttctccccttggtctttaacatgtctgctgatcaacctataatgatgaaatggaaaacatattttccgaagttattgtttaatttagggacaagaaaattgatatttaggaatttaaataatttgttcagcatctcaaagtgagctaatggtcaagaaggactttcatgagtcttaaggaaacaacctaaggatgtgatcatgtaataattcaaaacctctctattatccatcttcagggttagaccatgcaaccttcgacgtccccaaacttccccaggcccctacccctagatccctagctgtaactaccatatctgcaggtactgtttctagaaggaagtaatggatatttactgtttcatagcaaaccaaatctttatatttattgaaaatgtttgacagacatagatctatatctacatctatatctatatctatatctgtatctatatctatatacagatgcatatttacacatttatatttctatttttctttacagatacttaggagatgcacattagccaatgtgctaaaaattgtgatttgttgtatattatgtaataggcatacagctcagagtttatggttttgatttcgacagtgttttctgtggaatatccacaatttctataattaacactacagatatatttcaactgaaatcacgatacagagaagaattgaagtgttatataagtcatattctctaattttcctctcttattaacattagttctgttgaaactgaaaatacttataatgaatggctcatatgattacagcaggaaaataccaaataaccaatttggtattaaccaaactaaacttatagtaatatatacagttatataataatggttatttataggttctttctaatattacaaggtatgaagaaaaatgttgattctacaggttaataatgattcaatttatttggcaaaaattctctaaaaatacaggtctaaacatcctaattctagttctaaacatgtttttctcaaatataataacaattgtgttcaattttcatagtgtttgcttactataaccttttcagagcaaaaaatttgcagaggcactaaagatagacatttaaaattgtgtaaatattaaagttctgtatgaatgctttaaagaatgaaaattcaaaatgatttcacttttctttactcacctaggaagaggaagtttttgctccaaatattacctactaagactaggaatttcaaatgacaggattatagaattaaaggaacctcaaaggcctttggtcacagttcttggtagaattgtcccttggtatccatggggaattggttccaggactcaaatggacaccaaaatttgttcatgttcaagtccctgatataaaatggtgtagtatttgcatataacctatgtatatcctcccatatactttaaataatatctagaatacttataatatctaatacatgatttacatataaatgtcatgtaaattgtagttataatgtatcttttatattcatattatattttatcattttgctgtttttttaaaattatttttttctctcaaatattttgatccaaagttggttgagtcgaggggtgcagaactcacaggtatggagtgatgactatacttgaattaataggaaaaattccaaacaaaaccagaaaccaaatccttaggccttgctaattctaacaaacctttatccattgcctcaaatatatgaaagtagcacaaggacatttgctgaaggaagtatgtctctcatcattgccccgacttctcacatcagcctagcactctcatgaattttcaaaagatcggtcattacagtatgtttctaaaaccctttagcttctgctttctttacttgaaagggtcagaactgagtggaactgagaggactgtgaagggaggcttttcagtttgtcacatttgcttaattaaatgcattgtttctcaaactcatttgagcttaggccacagtaagtaatatatgtttatattagcactgtactctcatttttatgcaacatactctgtttgttaacaatttttattgctttattctattgttccccaatgctgaccactacccactaaattattttaagacttactaacatgttgttcactgaagtttcaaaaacactttcttggaacaaaaatttttctggaaataaatttatgagattaaatagcttgcccagggttctacattgggtgtggtatagtcatgaccctggctggttgacttggagcccgctatgttctcctgtttgtgaaatgataatgaaaaaaaaaaaaacagcaacaacaaaacaaaacaaaacaaaaaacttatatctgttccatatgctccaaagtcctattagtctgaacttcatagttctgttctgagaactaagcttggaaaatgcactgaagagcccttatctggtcctgtgtgcaggactagactcaggcagaagagcatcctgaacaaaccatgtattctgtcaccaacctccacttacctactaacctatggattcacaacaaacttacttgtctgtgataatctgtagcacagaacaaatttgtggcccttagagctaatagggaaatgagagccatggaagagagagaagttggttaagagacagaggaccatcaacacgggaaggattaaaggatccattattgttttcagtccattataccgaaggagtgagagggtataccttaagctgacagaaatgttctttttgcatttcccagagcttttttttatttaaataccagttatatagtcaactaaaagagatatgaaataccaccattctgacccaaaatattcagatcctccatgtggataattaaaagaaaaaggagaaagaaaaggaggaagaggaaaaggaaggggcaggaagggagagggaagagaaaacaggaaggaagagtaggagaagaagtaggaggagagaaaggagaggaggaggagaagggggaggaggggaggaagaagaggaaacaggaaggaggaaaagaacaaggagaagaagtaggagacaaaagagggaaggtagaggaggaggaggagaaagaggattaagaaaaagcagaaaacctctgtttagtaaattctacaagagatggaaaacatagcaatacaaaaaaaaaagcatgtgatacatgcttaaacaaatttaaagaatacagaaataatcccattctcaagagagagccaatgttcataaggttggtgtatattcttttgaactttttctttacttgtaatacatacatactttgaataccttgtatatacccaaacatgtctcctttactctgatacacacacacattttttaaggcaatcaaactatacttattgctttacaggttcctttttaaacttaaaaaatatatggtagacccatttccaagtatttacatacatggtagcttaattcttttttttttttttaattatactttaagttttagggtacatgtgcacattgtgcaggttagttacatatgtatacatgtgccatgctggtgcgctgaacccactaaatcgtcatctagcattaggtatatctcccgatgctatccctcccccctccccccaccccacctcagtccccagagtgtgatattccccttcctgtgtccatgtgatctcactgttcaattcccacctatgagtgagaatatgcggtgtttggttttttgttcttgcgatagtttactgagaatgatgatttccaatttcatccatgtccctacaaaggacatgaactcatccttttttatggctgcatagtattccatggtgcatatgtgccacattttcttaatccagtctatcattgttggacatttgggttggttccaagtctttgctattgtgaataatgtcgcaataaacatacgtgtgcatgtgtctttatagcagcatgatttatagtcctttgggtatatacccagtaatgggatggctgggtcaaatggtatttccagttctagatccctgaggaatcgccacactgacttccacaatggttgaactagtttactgtcccaccaacagtgtaaaagtgttcctatttctccacatcctctccagtacctgttgtttcctgccttttaaatgattgccattctaagtggtgtgagatggtatctcattgtggttttgatttgcatttctctgacggccagtgatgatgagcattttttcatgtgttttttggctgcataaatgtcttcttttgagaagtgtctgttcatgtccttcgcccactttttgttgggattgtttgtttttttcttgtaaatttgttttagttcattgtagattctggatattagccctttgtcggatgagtaggttgcgaaaattttctcccattttgtaggttgcctgttcactctgatggtagtttcttttgctgtgcagaagctctttagtttaattagatcccatttgtcaattttgtcttttgttgccattgcttttggtgctttagacatgaagtccttgcccatgcctatgtcctgaatggtaatgcctaggttttcttctagggtttttatggttttaggtctaacgtttaagtctttaatccatcttgaattgatttttgtataaggtgtaaggaagggattcagtttcagctttctacatatggctagccagttttcccagcaccatttaataaatagggaatcctttccccattgcttgtttttctcaggtttgtcaaagatcagatagttgtagatatgcggcgtgatttctgagggctctgttctgttccattgatctatatctctgttttggtaccagtaccatgctgttttggttactgtagccttgtagtatagtttgaagtcaggtagcgagatgcctccagctttgttcttttggctgaggattgacttggtgatgcgggctcttttttggttccatatgaactttaaagtagttttttccaattctgtgaagaaagtcattggtagcttgatggggatggcattgaatctgtaaattaccttgggcagtatggccattttcacaatattgattcttcctacccatgagcatggaatgttcttccatttgtttgtatcctcttttatttccttgaggagtggtttgtagttctccttgaagaggtccttcacatcccttgtaagtgggattcctaggtattttattctctttgaagcaattgtgaatgggagttcactcttgatttggctctctgtttgtctgttgttggtgtataagaatgcttgtgatttttgtacattgattttgtatcctgagactttgctgaagttgcttatcagcttaagaagattttgggctgagacaatggggttttctagatatacaatcatgtcatctgcaaacagggacaatttgacttcctcttttcctaattgaataccctttatttccttctcctgcctaattgccctggccagaacttccaacactatgttgaataggagtggtgagagagggcatccctgtcttgtgccagttttcaaagggaatgcttccagtttttgcccattcagtatgatattggctgtgggtttgtcatagatagctcttattattttgaaatatgtcccatcaatacctaatttattgagagtttttagcatgaagggttgttgaattttgtcaaaggctttttctgcatctattgagataatcatgtggtttttgcctttggctctgtttatatgctggattacatttattgatttgtgtatattgaaccagccttgcatcccagggatgaagcccacttgatcatggtggataagcttttggatgtgctgctggattcattttgccagtattttattgaggttttttgcatcaatgttcatcaaggatattggtctaaaattctctttttttgttgtgtccctgcctggctttggtattagaatgatgctggcctcataaaatgagttagggaggattccctctttttctattgattggaatagtttcagaaggaatggtaccagttcctccttgtacctctggtagaattcggctgtgaatccatctggtccttgactctttttggttggtaagctattgattattgccacaatttcagctcctgttattggtctattcagagattcaacatcttcctggtttagtcttgggagagtgtatgtgtcgaggaatttatccatttcttctagattttctagtttatttgtgtagaggtgtttgtagtattctctgatgatagtttgtatttctatgggatcggtagtgacatcccctttatcattttttattgcatctatttgattctgctctttttttttctttattagtcttgctagtggtctatcaattttgttgatcctttcaaaaaaccagctcctggattcattaattttttgaagggttttttgtgtctctatttccttcagttctgctctgattttagttatttcttgccttctgctagcttttgaatgtgtttgctcttgcttttctagttcttttaattgcgatgttagggtgtcagttttggatctttcctgctttctcttgtgggcatttagtcctataaatttccctctacacactgctttgaatgtgtcccagagattctggtatgttgtgtctttgttctggttggtttcaaagaacatctttatttctgccttcatttcgttatgtacccagtagtcattcaggagcaggttgttcagtttccatgtagttgagtggttttgagtgagattcttaatcctgagttctagtttgattgcactgtggtctgagagatagtttgttataatttctgttcttttacatttgctgaagagagctttacttccaagtatgtggtcaattttggaataggtgtggtgtggtgctgaaaaaaatgtatattctgttgatttggggtggagagttctgtagatgtctattaggtccgcttggtgcagagctgagttcaattcctgggtatccttgttgactttctgtctcgttgatctgtctaatgttgacagtggggtgttaaagtctcccattattaatgtgtgggagtctaagtctctttgtaggtcactcaggacttgctttatgaatcttggtgctcctgtattgggtgcatatatatttaggatagttagctcttcttgttgaattgatccctttaccattatgtaatggccttctttctctcttttgatctttgttggtttaaagtctgttttatcagagactaggattgcaacccctgcctttttttgttttccatttgcttggtagatcttcctccatccttttattttgagcctatgggtgtctctgcacgtgagatgggtttcctgaatacagcacgctgatgggtcttgactcttgatccaatttgccagtctgtgttttttaattggagcatttagtccatttacatttaaagttaatattgttatgtgtgaatttgatcctgtcattatgatgttagctggttattttgctcgttagttgatgcagtttcttcctagtctcgatggtctttacattttggcatgattttgcagcagctggtaccggttgttcctttccatgtttagtgcttccttcaggaactcttgtaaggcaggcctggtggtgacaaaatctctcagcatttgcttgtctgtaaagtattttatttcttcttcacttatgaagcttagtttggctggatatgaaattctgggttgaaaattcttttctttaagaatgttgaatattggcccccactctcttctggcttgtagggtttctgccaagagatccgctcttagtctgatggcgttccctttgagggtaacccgacctttctctctggctgcccttaacattttttccttcatttcaactttggtgaatctgacaattatgtgtcttggagttgctcttctcgaggagtatctttgtggcgttctctgtatttcctgaatctgaacgttggcctgccttcctagattggggaagttctcctggataatatcctgcagagtgttttccaacttggttccattctccccatcactttcaggtacaccaatcagatgtagatttggtcttttcacatagtcccatatttcttggaggctttgctcatttctttttattcttttttctctaaacttcccttctcacttcatttcattcatttcatcttccatcgctgataccctttcttctagttgatcgcatcagctcctgaggcttctgcattcttcacgtagttctcgagccttggttttcagctccatcagctcctttaagcacttctctgtattggttattctagttatacattcttctaaatttttttcaaagttttcaacttctttgcctttggtttgaatgtcctcccgtagctcagagtaatttgatcgtttgaagccttcttctctcagctcgtcaaagtcattctccgtccagctttgttccgttgctggtgaggaactgcgttcctttggaggaggagaggcactctgctttttagagtttccagtttttctgctctgttttttccccatctttgtggttttatctacttttggtctttgatgatggtgatgtacagatgggtttttggtgtggatgtcctttctgtttgttagttttccttctaacagagaggaccctcagctgcagatctgttggagtaccctgccctgtgaggtgtcagtctgcccctgctggggggtgcctcccagttaggctgcttgggggtcaggggtcagggacccacctgaggaggcagtctgcccattctcagatctgcagctgcgtgctgggggaaccactgctctcttcaaagctgtcagacagggacatttaagtctgcagaggttactgctgtctttttgtttgtctgtgccctgaccccggaggtggagcctacagaggcaggcaggcctccttgagctgtggtgggctccacccagttggagcttcccggctgctttgtttacctaagcaagcctgggcaatggcgggcgcccctaccccagcctggctgctgccttgcagtttgatctcagactgctgtgctagcaatcagcgagactccgtgggcgtaggaccctccgagccaggtgctggatagaatctcatggtgcgccgttttttaagcccgtcggaaaagcgcagtattcgggtgggagtgacccgattttccaggtgccgtccgtcacccctttctttgactcagaaagggaactccctgaccccttgcgcttcccaagtgaggcaatgcctcgccctgcttcggctcacgcaaggtgcgcgcacccactgacctgcgcctactgtctggcactccctagtgagatgaacccggtacctcggatggaaatgcagaaatcacccatcttctgcgtcgctcaggctcggagctgtagaccggagctgttcctattcggccatcttggctcctccctgcttaattctttttaaaggtcatatcatatcttatagtagagctatatcataattgttaactaatctcctgttaatgtggatattttgtttgaatgcaattgtttttacagacattgctgcaataaatgttattgcacgtatgtactggcatttgaatagagtaagtttcaaatagtggaattactagaccataagatttgtgcatttttaaatttggtagacactgaaaaaaaaacagtttgtttctgttacattttaatgagaaagtttcaatatttttaatttgtatttttattataaataatatggaacatcttttcagtgacttgttggagatattctgtttcttcttacctactcctgtactgtgcttaaaatatcctgcttctttagtctcagtaaatgacacttttgttgcctgtgtcagctgtttgtgtggatatgtgaagactcattgatctgcatacctccttaatgatcctgatcacaaagtgatgacctggtgggtcatagccttgggcttggaactggaccctactatgtgttatctgagtgatgtaaagagcaaagttttaaaatcattttttgaatattcaaccattcttcctcaactggataatttccattgctttttgaaaggataattttcactacatgattaatagtcagaaaacaaaatttataatataaatataattatgaaaaataattatatttatcattcagttaaagaaaaataacattgtcatgatttttgaagttcttttaagtgtctctcaacatcacattcttttctttcccaatacagaaattagtgttgattaattccttgcttccctttctaattttgccacattaaaaaaaatccaatcaatatattgtttagtttttcatgttttgagcattatataaatggaatcacatttttttgcccctttagtatcctgaaatgaagccatgttgtgatgtagaactagtgacttattttttactgctatgtaatattctattgcaaatacatctatttattctatagctggcatatgttaggatttttccattttaaaaaattgtaaatagtgtagcttgatcatcttagtacatttttcttgatacacacatgcaagataattctctagggagcagttctcaatctttgctaaacgtgagaatcattgagagattaaaaattctcatgtccaataaaccaataaaatcacattatataatggcaggacgtgacagtaggaccagcttcatggacatgtggccaatgtagttacataggccctgtgctcagaagaatcccagatctggggtttaatgctctgcagtcattgtcgaaattcttaataattttcttttgcttttgtttttgaaattcaatgaaataataaagcacacaagaggtggcttggagcctcagcacatgtgtgtttctgtgtcttgccatttcgcatcttcttaggggcaagcaagttctcagctgcctgctccccatcctctgatgctgggccctgcccaacaccccttcacttcgccatcctgcaactgctgccagacatttgtctattttctaaaaagtgatattgagccttccaatccacagatatatatttttttctttcctgtcttataataaatttttgttactttcacaatgaaaagtaatttctaaataaattttttcataacttttgctatctataattatttctaggtatggcccaaatattacaattgctattgaaagtcatattttctcaggattatactgtcaaactcttcatggttgaactatagaaattcatttgatttctacacataaattcatgtgtagcaaagttgttaaacactcatagattttgacaatttatggaattattttgttcttccttttagctaaccatatactcgtcaataatcacagttttgtttcttttgttcaatgctcatgcttttttttaatcctccccaccacttcctataacatctaggacctacagaaaaaaagtgaaatataaatggtgatagtgagcacccttgccttgttcctgatcttgaagagaattatctcatcatttaccattaagtctgacatttgtcacaagttttttgtagatactgcagattggaataaagaagttatcttctattcatggaatgcaaatcacttttaaacaacaaatgaatgctgaattttattaaatgctactatacatttgaagatctcatctgaaatttgttcagtactttttagtcattgtcttgtggtagagtgatttgtcatggttctaatattgttagactatcagaaatagaactaaagtattcatttaaacacattcaagaatctctatttgtacaaaaaggaaaaaaaacagacacaaataaacccaacttattcattagcaccatgtcttttcccctttcacagacaaattttccagaagagttgcctgggtttattgtttcaatttccttttctctaacaggttgatccaccctttccagtctggcttctgggtatagatccactcacaaaagcagctttcccataggttatcaacaacatccatttcagagggcctggaggtccttgtcttatttggattttaagctaccttcaagaacaattgatatacttttctttcttgatatactcccctcacaccttagctcctattcctctgatcaccctgaatgctcctcttatttctactttgtaggcttatccaattggctaattaatatttgtgtttcaagactcagctgtagattctctactaaagtactgctataatcttccccaaggagatcccatccatgcccatagcatcatcacttcttataatgacttacaatcttcaaggagacctcttttctaagattccaacccaattgcctgtcctcctacttgatatattctttaggattttgagattgtgatataacaaataagctccagaagctcagtggctttacagaatggaagtttatttcttgggagcattaagtccaatcagcattaacattggtcatttagaggactagcctctttcctacatgcagctctacctcagcataggacctctaagtcttccctactcagcagaggataggaaaataaaaaatgtggtttgcctcacagtcataaaggagcattttatggttcgatggtggcaacagtgcatatcacacacactcatggtccactggccccaactcagtcacacggccacacttatctccagggagacagggaactatagtctagctttgtgccaggaggaaaggcaattgtaattgttaatcaacaaataagtctctgcaacaatttacccttcctcttagcaaatttccgttgcatttttctcttcacacagagaatatgcttattccttctccattggagacatcttaatgtttttcaaatttttattcagcatcagccgcgaactcaaagccctgaatgttaaaagatgtgcaagctaaatgttgtggcaccttgtaatagacaggaaacccactgccatcttcccgacacagacaccaaacactaacacacccaaacccccactataaacctacatatagtatcagggacagcaaaacctcaaaaaaaaaaaaaaacttctattcaaaatcaggaaaaatgggagaacaataacacacagtgagatcctatactataggcattgtgcagcctctctggcagtgtggatttcagtaaggagaacctgaatcagatatctgtgaagaaccaccttctgtggctcctattttatcctctgaaaggttcttccttgaccgtatttttccacggccatatctgaaataggtttggcggagtacaccctcctcggggaacatggaatgttcatagccaaatcctgttcatagagtttgaaggactgaaagttgttttaaagtttaacagtcacagacttttgcaagcagactggtggctcctttggcaatataatctcttaaaaatgtgttagatttctcatgtacttgctttttatcagttacatgtgccagtattcacaataaaaaatttttcttgacttagttcccaagtttgccttatttctttccttcctcacctctgtgcctctctctctctcatttaataatttaagctaatctaaacaatagactgtgtaataaggtaatactcttaatctgagatttgctccatcattgaatcaatttatttaacttagaaatactaggccttttatgactggagatattttcctttgttttcttcaactttttttttttaagttctgggatacatgtgcaggatatacggtttgttacataggtaaatgcatgccatagtggtttgctgcacagatcatcccatcacctaggtattaagcccagcatccattagctattcttcctgatgctctccctcctcccaccagccacctgacaggctgcagcatttgttgttcccactgtgtgtccatgtgttctcatcattctgctcccacttataagtgagcacatgcagtgttcggttttctgctcctgtgttagtttgctgaggataatggcttccaattccatccattttcctgaaaaggatatgatctcattcctttttatggctgcatagtatcccatggtatatatgtaccacattttctttatccagtctatcattgatggttatttaggctgatcccatgtcttcactattgtgaatagtgctgcagtgaacatatccatgcacatatctttataatacaatgatttatattcctttgagtatatacccagtagtgggattgctgggtcaaatggtatctctgcttctagatccttgaggaattgccacactgtcttcacaatggtcgcatgttagttttgatttgcatttctctaatgatcagtgatgttaagctttttttcatatgtttgttggccacatgaatgtcttcttttgagaagtgtcactcctttcctttacccactttttaatagtgttgcttgttttttttcttttcaatttgtttaagttacttgtagattctggatattagatctttgccaaatggaaagattgcaaaagttttcttccactatgtaggttgtctgttcactctgatgatagtttattttgctgtgcaaaaggtctttagtttagatctcatttgtcaatttttgcttttgttgcaattgcttgtggtgttttcatcatgaaaattttgcctgtgcctatatcctgaatggtattgcctagattttcttctaggattttcatagttttgggttttacatttgtctttaagccatcttgagttaatttctgtatatggtgtaaggaagggatccagtttcaattttctgcatatgctaaccagcactccaggcatcatttattaaatagggattcctttccccactgcttgtttttgctaggtttgtcaaagatcagatggttgtagctgcgtggtcttatttttgagctctctattctcttctgtgtatctatgtgtatgttcttataccagtatcatactgttttggttactgtagcctcacagtatagtttgaagttgggtagcgtgatacctccagatttgttccttttgcttaggactgtcttggctatttcgctctttttttgctccatatgaatttttaaatagcttttttctaattctgtgaagaatgtcaatggtagtttaatgggaatagcattgaacatataaattactttgggcagaatgaccattttcatgatattgatttttcctatccatgagcatggaatgtttcttcatttgtttgcatcctctctgatttctctgagcagtggtttgtagttctccttgatgatgtctttcacttcctttgttagctgtattcctagatattttgttctttttgtagcagttgtaaatgcgagtttgttcataatttggctctctgcttgtctgttgtttgtgtataggaatgctagtgatttttgcacattgattttgtatcctgagactttgctgaagttgcttattagcttaagaagcctttgggctcagtcaatggtgttccctagatataggatcgtatcatctgccaacacagatagtttgacttcctatttgaatacactttatttccttctcttgcccaattgctctggccaaaacttccaatactatgttgaataggagtgctaagaaagggcaaccttgtcttgtgtcactttgcacattaatcttatatcctgagactttgctgaagttgcttatcagcttaagatgcttttgggctaaaacaatggggttttctagatacaggatcatgtcttctacaaagataatttgacttcctcttttcctatctgaataccctttatttcgttcccttgcctgatttccctggccagaaattccaatagtatgttgaataggagtggtgagaaagggcatccttatcttgtgctggtgttcaaggggaatgcctccagcttttgcacattcagtataatattggttgtggatttgtcatagacggctcttattattttgaggtatgttccttcaataactagtttattgagagtttttaacatgaagcgatgttgcattttatcaaaggccttttctgcaactattgagataatcatgtggtttttgtctttagttctgtttatgtaatgaatcatatttattgactgggctgtattgaaccaaacttgcaccccagacatgaagccaacttgatcgtggtggataagattttttttgtgctgctggattcggtttgccaatatttaattgaagatttttgcatcgatgttcatcaagaatattggcctgaagttttcttatttttgttgcatctctttcaggttttggtatcaggatgattttgtgctcatagagtaagttagggaggagtctttccttttcaattttttggaatagtttcagtagaaatggtaccagctcttctttgtacctctggtaggattcaggtgttaataccatcttgcttggtaggctatttattactgcctcaatttcagaactcattattggtctatttagagattcagtttcttcctggttcagtctcgggagggtgaaggtgtccaggaatttgtctatttcttctggattttctagtttatgtgcatagaggtgtttatagtattctgtaatgtttgtttgtatttctctggggtcagtggtgatattcccccttattatttctgattgtgtctatttgattcttctttcttttcttctttactagtctagctagctagctattttatctaaaaaaatggctactggatttattgattttttgaaggattttcatgtctctatcttcttcaatttatcttggatcttggttatttcttgtcttctgctagctttggggtttatttgctcttggatatttttcaatcttatcttttactatttgggacctacaagtagtcggctttttcaatgttaggggatccttattttaatgcctctaatctttgcttgacaaccaatttctacctgagctcatgtctcttttgtaaaaccctgctcaagcagccaagagtgagccattcatactatcactccagttctttcaaaccaccacatgtagtgctactggctgggtggatatctgatctcctttgcaaattgtaccaaataatttgccaattcacaatttaaaaacggtctccatctttccagcccccaataggcagtttctcaccacctgactgctaagacaattctccatattttaaactgtggcagctgccctacttcaaggtgtcaatttttatataggctaggcatcactaagccatcaccaataacacatcaaataccagtaggccaaaacaatagttaatttctgactcacatgaaatttaattccagagggaagaggtgggatgggttgagtgagttagaggaatttaggtgttatacagctatttagtgattccaaatgtttctaccgtatggccacaccctcttctaagtttacagatgcttcttcattcatcctgcagattcagaaaaagacattacactggagatttttaggggccagtcataagtgcattccacatgtacttctgtttctacttatctgtggggaggctgggaaatatagtttagctcgataccttggaggaagaaaagtgaatttggtgagtggcttgccagtctttgccacagtatttccaacaaagcatgtaatctgtctccctaaaactagtcctatttaattatcatttgtaccactctattatagatagatactgaaagatccaaaattatttttgaatatggccagtacatataacagagaacaaagcataaagcaatgacttttgtgcagtagtttatctgggagcacatgtaaaggagatggggtgtcaagagtcagtaaaaagatgcaatactgagttgttttctaattcaggtaactgaagttttcttctttggggaccttctaagatgctttgtgaaatacatcactgaactttattcataggagaagaaaggggaaatcatttgacctttggatcctgtccctcactgatttggggtgaccccactagccttgattccctcaaactcgcatacagtgtatgcatgagtgctgagtgggtccccacatttcgtgcttcagtggcagaaaagtactgggaaaagaaaaatgaaaagcatggtacaatgtccaagatgaagcactcttaggttgcagctgcataaaaaaagattaggcattctatgaagaattttgatggtggggaaggaaggcaaattcatatccaaagtaagtataaattctagttggaaagcatcactacctctttcaagtagaaaggttacggtattataaatctgccatcaacctgctaaaataagatcttggtataggtatcagttgttgctggaaggtttgccattcagcattggtagaacactaactgatcagccttatggagaggaaatccattctgtcaggcccatgcatagctgccatccttgccaccatagctacattcttcaagctcactgcaaaactatggtcatggagggtcttctctgtggtagatactctctgctggcaaaaatctgagacagaaaaatttgcccacgtcttgccactaccatgggtacttccacaagtctttttccctcattcccttttctacagtcttccaagtctgctgttttttttaatccctttgaccaagcaatttaccactgaccatgagtcttacttctagccacttgtctttccatacaaagtgaacagtcaagagtactgctcatgttctgcctctgggaaggatttccttttaccactggcttctagagccacctctgtgagtgtttgtagtcatctgtgcatggacagtaaacactgatatactgggttcgtctttctgggaatcatttacttaacagatccgataatatccaataggtgctaaatttcaaatggcaaggagtattctactgcagatggaatggttttgcttcagagcccaaggtgtctgtgttgtaactctcctattaagttcttgccagagactccatataccaacctgagagcttgaatgagattaagtgtataaagtgactattaaatagcaaatattgtgtatatgttacacactgtgcctttatttttatatttttaacttttattttaggtttgggggtacatgtgaaggtttgttacgtaggtaaacatgtgtcatggggatttgttgtacatattatttcatcacccaggtattaagcccagtacccaagagttatcttttctgctcctctccctcctcctccctcccccatcagggagaccccagtgtctgttgtttccttctttaacactctgcctttaaaaccattatgttgatttggattaagaattgaaccattaggcttcttttatttgatgccttacaaagactatagtgaatactgctacacatttttcagaatttattttttatgttttgctttttccccaaatttatatattttttaaattgatataaaaattatatgtatttaccatatgcaagatgatgttttgaaatacacacacacacacacacacacaaactgtggaatggttaaatctagctaatttacacacacataacctcacatagttatcatttttgtggtgagaacactttgcattcactctctcagcatttttcaagaatgtaatatatcatcattaactatagtcaccatgttgtacaatacatctcctgaattttttcttcctatctaactgtagttatgcatcctttgaccaatatctccccaacaacccttgcttttaataatcatccctctattctctgtatctatgagatcaacatttttagattccgcatacaagtgagatcatgtggtatttgtctctctgtgcctggcatttttcgttcagcacaatgttatacagtttcatccatgttgttgcaaataaaaaaattcatttttttccatggttgaatagtattgcattgtgtatgtatatcacattttcttaggttgattccatatcttggctgttgtgaacagtgttgcaataaacatggaatgcagatatatcttcagcacactaatttcacttcctttggatgtatgcccagcaatgggattgctaggtcatttggtagttctagttttaatttttagaggaaacttcatactgttttccataatggctgccctaatttatttccaccaacagtgtgctaggggtttctatattaaggttttactaaagccagctggttccccaactctattagtaacaatctttccactattaatgaagaaacatggtcacaaagacaagcccaaactattgaggagtattactggacattaaatttttggttctcaaatctggctaatcctcagaaatatatacagagtgtgttgaaaatataggtatttagccctaaccccagtaattctaattcagtaggcctgggatagagttcagcaacatgtatttaaaaagttatccaggtggttttgattttcaagcaagtctgggaaccacttctctaatccacatttgggaaaacccagtcaccagccataggtcccagatcctcttttcacttacacctctcagggaataagaaaagtctgtgctcagaagggaaagaccaataagactaataccatgcagctcccaaggtggcctgcttcactccagtgcccaaaacaattgttggtacacattagccactcaataagtagtgaatgaatgaatgagtaaatgaatgaaagtcaaccatagttctatggcagcactgttcttgaattcaatagcttttccttgctttattggaagtatcctaatactgcttctctatttagagcctcaattctttatgtttccactcaagctggaacttttaattcaaatatttgagcaaaagaatcaggaattaacaagaccaggctgctactgctcactttaataaaaacatttcaagctccttgtattttccaacacttttcctttttatagatctgctctcaaaaagtttgagtagtaggaaataattttacagttgatccttcagtggtgtcatcattgcaaataagcaattgatcctaacacatttttgctcttaaatgtgtgcattcctttaatgactgatatggttagccctatctgtgaatgacagaagattgttcccaactgatttccagaaccagctggcttttgtgaaatattaacataaaacctcctcaaaatgtatatagtctttttcaagaagctttagaaaagagcctttccgtacctgtttctaccatttcatttctttttatagccatacttctcacccatctgtctatcgatccctcatgttagatgtcaagatgctagtaagattggtttattcatcttacttgtctgcattcaatggatagatgatttatttggctgcatttcatcctgccttacaacatttcatctgtctactcccagtgaaggtctgggtttaaaaataacattccattagcgagcatttttatagaaagtactttgaatacactcatttatatatggaggtgcatgatacatagtcttacatttttttccttaagtacataaaattttaaacttaattttaccaaaataatgcaaagactgtgtaaaatgacttaataaaggttcgaactcacttttgtaattacatgttataatttttactattatctgatcactgactgtctgaagaaagattacagactataaataaaacactgagctaagtgaattgtgaaagacatttcccctgcaaaaactcctctctctctctctttctttccctgtcttatgcacacagatatacatacacgtatacataaatgcacatacatcaccttctagtatagccaattcaaataaattagtatttcaggagctttatgttaagttttggctttaaataaatcacttcatctagccaaaaccactgactttttcttggtttctacacaaaactctaattcaagtctagtttccttcaaattcagtccaggtgctaaaaaagcttcttggttttccaaggaacattcaacagaatttctctactctgtattcatatttatatcatagcctctaaacagtccagtatttggtattttctggattaaaatggttccatggtgaatttgtagtccattggattcatagacattcacttataaatgtttgtttttcctcttagaaataagtgattattccttaaggatcttgttttttattatttgcattgttttgaattctgtagagaacaggcatatgtgttttaagttagcaataaagagaataataacaaataaactgtttctttaaaattactttaaataccatccaatgtaaaaatgttgatttataataaactctacaacttttaggttttatgctatttaatatatacacttagaattctagatatttctttgggttgggtcctcagggaaaagtcagtgtatttaaccattattagctttcaaatttaaaatataaatagtgccccttcttccactctccttcctcagcctgactcttacatttttgattaaaaacaataatcagcaacaatgactctagaagtcaaattctgtgcttggaaatgtaaatagaccttattacagagcacagccatagagaggcaacatagcaccaatgtgtctgggttcaaataatttttccatcatttacaagataagtaaccataaacaagttacttctctcactttccttcaatttccagtctgtgaaatgaaaatcacaataaacatttctaactaagaatgttggtacaaaaattatatcagtaaagaaatatctgaaacatagtaaaactcagtaaatactactttttatcacagattttgaggggtttgaaaaatcaggcaaatcaatactttttgaataattatgatgttaaacatgtaatatgggtagaaaatttctggaagatctaaggcatattttcttagaataagtgacttcttaagtatggtgttatctttgaataattttagggtagataatcaactggggctattagttgcaaacttcattgttcataagaatcacatggtttccagttaaaatccagattctgattcattaggtctggggtagggcctgagatatgcatttctacaagcaactaggtgaggctgatgctgttggtctaaggatcacattttaaatagcaattacctctaaggatcacattttaaatagcaattacctcaacaatttcttgaggacattttaagaagacatgaatttactatccaatctcatatacaattatgcactgcataatgatgtttctgtcaaagtcagactgcataatgatggtggtcccataaaattataacatcgtatttttactgtgttatactttgttatactgtgttttaccttctctatgtttaggtacacaaataccattgtgttacacgttgactacagtattcagtattcagtaacatgctgtacgggtttgtagcctaggagcaacaggctagaccatatagcctagatctgtagtaggctataccacctaagtttgtgtacattctctgatatttgcacaacaaaatctcctaatgatgcatttctcagaatgtattctggtcctgatcattaagctacacatgattgtacataccttcctgccgtctactgggaaatagactaacctgattgacatgatgcactttctaatccaatgggcttgaaaactggggcatttacatttaggacaagttcccaggtgatgctgaaattgcttgtccaggtaccacactccatgaaacactggcttagagtactcattgattctcttcggaaaatcaggtggaatctggcaatgttcacttacttaaatcataaacatagcatacactactgttaactccataaggagaacttcaacactagttcctttgagataccatcccgatgttttcgaatttgcttaccaagtcaatggaacaaaagatctcactcataagtgagagttgaacaatgagaacacatggacacagggaggggaacatcacacactggggcctgttggggggttgggagctagtggagggatagcattaggagaaatacctaatgtagatgatgggttgataggtgcagcaaaccaccatggcacgtgtatatctatgtaacaaacctgcatgttctgcatgtgtatcccagaacttaaagtatataaaaaaaactcaagaacttccatttatccccacacaataaaacatccccagactcaagagaaagagaagcattattttttctattaattaaaaataaactattactatattccagaggcattagtatcaagattatcatgttataaacatgaaaaagtagacttggataactggaagaattcccattggccccacaattctactgtttacatttgataacaactgatgggacagataaaagtcaagagtcagaaaacatctgaacactgagtgtcatcacttgattttcagcatcaagcacactgtgtttagaaaggagtgaagaatttttgcttcgcactgggtaaaattagacttggaagcaaagagcaaccaacagatgtgtgtcagggagagatcagctggataaggttagttgtttaacatctaagtcaaacctgaacatatttgagtaagtcatattttccacagtaacttttgcaactttagaggttctttggtcatggcagttggaatttgcatcagaacttcgcaaataggaaaatctcccttaagttcactctagattttcctagatttctccaaaaagcagcaaaaaaaaaaaaaaaagtcagactcagctacggagttagcctatgaggaatgctccaaccttgctgatggtatacttgggactatcctggaaagcatcagtctttagaatagaggtggagcctatagatgagatccacctgtgcaattagctttacatttgctgtcacttctgatggaaagcactaagacaatcaggtgtttccctttgagcacactactaccttcctcaaagaaactacagaaatagtgaatgactaatgaccagaagcatatcaagaaaacattacattaatattaatagtataagaatctggacaaagtcttgaaaataattatcccatttgaccagctgtaaagaatcttctcatggatctgcttgccactttatctccacattgtaaaatgatgacatggagaaaactgaagctataaaagatgtatcttaaaaatggagatttaataaacatctaaagatactgctgttgaagctacattctgactactaatgctagctgacttgtctttcgtttgctcgagctgctgagacctaattgactgctatgtgtcagacattgttctattcattttatgtggcttaactaatttaatttttacaagcaatatgtgaagtaggtgctctttcttttacccaaaagaaaacagaggcgactaaaaattagtaacttgtccaagtcacaaaaaaagacaatagagccagaatttaaacatagctgtttttggcaccagaagctgtgattttattcaccataatatactgctctcgtctaatgatataaatcttataattgtcaattgattataaatgttacatttcacagggaacacaggaatataataagagactatttaaaaagtttgtttgatgagaggcaatttgttgcaatataaagaagagcctaagaagccagttctatccctacctccaccaggttgtgtagaggaaattagttatcttctccctagagctcaggtttctcacatattaaattctagtaaagatttcaaagaaatagatgatctctgatattagatgtgttctgatagtcttggattaggtaactgaggctaagttcagggccatttaagcaaactccagactgtgtatgtggccccctctggagtgactatttatttaatattaaaaagacaagtagcccaccaataactttcctttcctaatactatactaaaattttaagaaagcctgtattatttctttctttgcccttgaaaaaagtacttattctttcagagagctaaattgagatttgggataaaagagttttctctagttccagattaccttttattgctttgttttaaaaattctaaatagctaataatgtgtccatattcaataaacaatcataataaggcacgtttctttgcttctagtacttacgtgtttgactctataaaactgcatatttttttagcaaggaacacaataattttcacctaagggacattcaaaaatatgatgtggaacttttgtcatctacaaatccagtatgttggtcattatttgccactttgaccaggcactattgtaaaagtgtgtgagtttaagtgaatgcgtgtctgttggctatgtttttgtaagtatatgtgtatagggaatctttatctgttttaatttgggcaacttaaaattagattactgagagagacccagcttcccctcatctctctcaagatttgactaagagaggcatcatatctggctgcaacttctacctttgttggctaagatttcaaccagatactctaaggaattatctggaagattttatcttaggacctttcaaaattcaaaattccctcaagagaagagacatggaggagtagttcctaaagatgcagcccattccagtggagacaaatgctggctttagtttcaccactaggtttacttgcactcaaaaattcccaataaaatccagctggtttaaattttgtctgcagacctgaaacactgcatatttggctaaggcttcctattttgcagtaaatgcttcacagggctataatctggaaatactgaagtgtacaaaccctcaacagaaacaacaggagaacggctgtcttctaccttcattttctcctaactctactctaaaggcataggtgttgttaaggaaggggaaaaatccttcattgaacatgaaatgttgtatgaatcatcatttgactacctttgttgtttgctcaaagccaaaacataaagattaaagagttgccattgatgagtgagacaattcacattttggcattactagagaagaaaggagcatttaagatcatggagggaaataaaacaacaaaacaatactgttgcaatttgaacaataacagccttcagtacatgaaatcatagtattatcttttccattttccacccttatattttcattggcttcatacaatcctcttgttgcctataattggggatagggttagtgccaaagctgcataaaacaagcagcctttcctttatactttctttgcatcgtgattgtgtatgtgaagtcataaaaatcatttattatgagcatgtgtattcttggcttaaagagccaagtattcttgtgacaacaatataatagcatcagatgtattgccataaaacaccatatgtgggcacttaatagttactgccctggcacctacatgctgggatatcatcttaaagagggactctttagaaaaaaagaatgtttggtacttagacaaataaagctccttggatgagataggtgagcaatgagtagacatttgtgaagaatccattgatgatggcaacggttcgtcttccattagtatcagattttctcaacccatctgctggagttcttttcatgggtccaagaaaatcctttacaacattgcaaacatcaataaatatctctcaggctaaaagttgcaagaatgttttaatgtcatatttacagctaataagctataaaatgagaacaacgtaattttcattctgtgcaaccattactctttggaaagcatttatttagggtatgttgtacaaatcattagtaaacaaattagttctcaaactagataaaagaatgtagaatggatgaaagccactgcatggcacatgtgagcccttggtggtgtttcgagcctctgtgacagacactgctccccactgtctctgtcctttcttctagcaatgatttcccttggttgctgctgaagctagagactaagctttcccaagcatcaatgcacttcaagtttgccataactctgggactgatgttctacttctgcattagcacctgagtcaggtggccagacattaactgtagacacatgctagtgtctttcaaaaaaaactcagttgcaaaggaggccagagtccactagttcctgagtgcatgtctgctttagttaggagtgaaggcgatctgaaacaagaaaagccacataactctgtttgctgagttttctcagagggcgactcatcttagtgatacactgctgtgcgtcactggtgtctgtgtaggaagatgctactcttgatgttttgagtttccaggccagacatgattcaatccctgaatctctattcactagctctttctagtataacagacagtctaaaacttacaatggtattttgttgaaagaacatatggtagctattacattgaaaatgtacactaagcatatgtctacaaccctaatagctacttccaacacttctacacaactgcttcgactcagtcaatttctttcactgttctttggcccaaactgccattccagcacccctaccctaaaatggaaatattattccttttaattgcttttgttattttaatactgccaggtagctgaaagggaacttttgaggtggtaacatctcttactgatccaaatatgtttttcttcagttggtaaaactggcttagcagttaccgtcattatgtctggttcttctctaccagcttatttttaaaggagttttcgtaagaaacataactccccaacctctccctcttcctgttcttcccccagctcccctcactaattaagtatttcatttccactagcccattataatgttgtttatgatctgatttctctttctctttttcatttccaaaatcatgagttttcccctttctaccaatggtctacatcctgactgtatagatatatgctttacatgtttttgttttattattttaaaaattttatgttaagttcaggggtacatgtgcagatttgttatacaggtagacttatgtcatgggggtttgttatacagattatttcatcacccaggtattaagcctagtacccattagttatttttcctgatcctctctctcctttcaccctccactcttcaaaaggtcccagccagcatgtgttgttccctctatgtgtctgaccatatattgaaagggtatagaaaagtatttgaaattatgaaagcctagtacttatctctacttttcccttgccctattaaatcaaaacgtacagcaatagaacccagaaatctctcattgctccataggtaatactaatgtgtaaccactagcaaaacataatttcttactttaaaaaaaatagctcctgttgtatgtttaccctctgcaagttaccttacatgccttgcctcatttaatcctcacaaaaaaacagtaaatattattatcctaaaattttctaggatagaaaactggagcatcaatgagtcagaaaaaagaaggaaaaacaaaagtacaaattttagagcaaggtcttcaatccatgattggaagtcaaaggctgacccctttctactatgctacactactcctcactccactctattatctatgtttactagtatttttatttctaattctcattatgtatttgtgtgtatatgtaaagtgacaaatcagctggaaaatccacatttacaaaaggtgctaatacctcatatggtaatgcagtactgtaagatgtttatgaataaaaggaatgtggccctgactgacgtggaataatttaaatctcagtagagataatgatgctgcatcccatacttacttttgagaatatggtggactttaaaataacactgctgcataataaataaggagtgactgcaattaatgcatacctcactgcctaaggtttcccaaaagagaagggaaagccttcctatttccaaggtgggaatgttcttcaacgctctcctgacctttctccagtttcctcctttctcacctttctttaaacccttttcactttttcttctcttttcacctgcaagtctattgacaggtaagtgagagaagagaaaagaaaaagctagtatttattaagcacctgcaatctgtcaaaaattttcattagtggtatattataacccccctgaattagcttttgctatgttatacactaacatgcaattgtcaaatttcagtggcatacaaaaacaaagattgatttctaggtcatgccacatgtaggcagctgggttctgcttcccatttctagactcaggctgaaggcacagttgccattgggaacatgccatttttatggaaaagataaaaacaagcaacaagatcactcttaaatatctgcatgaatataatatatgtcctttctttcttacatttttgacaaatgcaagtcaaagtgagcccaatatcagtggagtagtaaatattgacctcccatagaaagtagtgctctaggccaggcgtggtggctcacacctgtaatcccagcactttgggagaccaaggcgggcggatcacgaggtcagcagtttgagaccagcctgaccaacatggtgaaaccccgtctctactaaaaatacaaaaatcagccaggcatggtggcgagcgcctgtaatcccagctactcaggaggctgaggcaggagaatcacttgaacctgggaggcagagattgcagtgagccaagatcgcgccattgcactccagcctcggcgacagagcgagactccatctcacacacatacacacacacacacacacacacacacacacacacacacaagtagtggtctaactcacagggcattggatggtgcatgcatatatttttacagcaaaatagaagtgaatctttataaaaaaatataatctatcgcaataccctttttatataggggaaacatgaggctcagaggttaaattaactgtccaagagtagtgcatctagtggacgactcatttaagattgtagtcaagttttttctaattctacagccactgttcttggatttgcatagccaagttgaagagaggggagacagacttagttctctcttctattattttttaatctttcattccaaatattttctaaaacatcacgtcaccttaaggatctaggaataatctttgatttaatcctcttcattttttcatattaaataaaactctacattgtctaatgcttaataatgatacaattttttgagcacttaacttgtgccaaacactatttcaaactctcttcacatactgttttatttaattttgaaccataagttttgtggtaggcatcatatcactttaaagacaaagggctacacatagtggctcatccatgtaatcctagagctttgggaggccaaggtaagaggattgcttgaggccgggagtttgaggccagcctgggcaataatagcaaggccttgtctctagaaaaaataaaaattagtagggcatggtgacatgcccctgtagtcctagctactcaggaggctgagacaggaggattgcttgagcccaggagttcaaagttgcagtgaagtatgattgtgtaacctgggcaacaaagcaagaacttatctcaataaaaaaggataaaaacattgaggaaaaaatctcaataacttgcctaaaatgactgactgggagtgaagtagagctggtttttaatccatatctgatgttaacacttgtgcttctatgctctgcatcattctgctttctaatgaaaatctctgttttaaatatatcctacacttctctcttctcgtctccagcttctattgcctatgtttagtttttatcttgttaagcctaaatttctgctgttgctttctagttagatttcactcatgaaaccaacctatataccaagactagactaattcttaaactctgccttgatcacttttgtgtgcagaagacattcattgctctcccttcttcctactttcatccttccctcatataaactccttcatctgatttccaaggacacccagagtgcaaattattcttatttcccactagtcctcaaagtgtaccatttacctggttgtcccttattgattcaaccttgctttatttacatttttccccttactggaaactagatcaagaactttacgggagcaaggtcatgcatcattttatgaatatctctccatattgattgtcattatgctagctttgaagtaggaagtaattacttacataggtaacctttacttgggtccaaatatggtgcttttcatcacattgttatgtggacatttacaggtaactaggaataaatgatccatgaattcatttctggttctgctgtaatgggtctcctgaatagacagcagattctaaattctccatatctcatggggacatgttgggaaattgaagaatgccagattaactggcagcaaaagtgggattgatgttgcatcacatcgccctctctaagcaacaataagaatagcacttgaaaggtcaggcatctttcaaacctcagggtgaaaagtttgcttgaacacatggacaaatagaggggaacaacacacttgggggcctgctagagggtggagggtgggaggagggagaggattaaaaaaataactaatggatactaggtttaatacctgggcgataaaataatttgcacaacaaacttccatgacacaagttcacctatgtaacaaacctacacatgtacccttgaacttaaaaattaaacaaaatagaataacataatataaaataaataactgaaaaagaaaaaaggaaagaaaaatttgcttggctcccagaaaaacatatgaagagaaattgtcgtacatagcgtttgcatatacgtgtgtctagtagaggtaaggattataaattagtacttacatttatcaacacacaatgttttcagtgtggtgttctcttgccttccattgactaagcaaaaataaagatcctcaatgaacatcttatgcctgcacacattttataaatccttgccatttaatcacatatatccatgttttccaatttgttttcctggattctaaaatatatcccctggagaaagtaaatttaggtaatgtatgccactatattatgtcaaaaaaactgaaaattacttgcaactaaaatgcatatattacatctaacccaaaattttctaaagtcatttacttatgggatcttttgtttgcctaacccataaaagtattctgtagaaccagtgttttatggaacataattctaaaaactctgcctcttctaaaaaagacgttgaatttactgtgtccccttgaaaatagagaatgacagatggttctacttgagtaaaatggcctgagaaaatctttcccagaaggtggtctttaggcagacacctgaagaaagagaaggagtctgttctaggaagaggcaatagcaagggttgagtgctccagcagtaaagaaaatgtttaatgtgtttggcaaactaaaaggaagtaagagaaagaggaaggaaggaaaagaggcaaggggggaggaaagaagcctcttggtggctggaatgaaatgggcaaagacgagatttaatataccaaagagattgctagagtttagatcatgtgggacttcctagacatgatagaggctttaggatttcatttaagttcagtgagaggctatttaaagatttgaagtaggggaaattaatgatttcatttggatgtttaatagataatcctgattgctttccttgtagtcaggcagaagtgaaaacaggaaaaaagttgagattactgggggtatttattgaagcacctatgctggaatatgatgatcactttagctagttcagtgcagtttgcaatgaggaagaataaagatacctatttatgtaaaatcaacaagacaaactggctaatgggatatacgattgaaagaagggaaaaaatctaggataatttccagattacctgaataatatagatgggccatttcatttactgagatgagaaacacagtgagagaagtaagtatagtaagaggaaacctacatttagtttagaacttgttaaatatgagatggttataagatatgcaagcaaaaatatcaagaaggtagcttgaaatgaatctgtagtttacttaaaatcattggaaaactgagatcactcagtaagattattaggtttcttcttacttaaggggaggggcaggactgaatcttattaaagggaagggccaggactgaactccagcctttagaagttgaagacagcagaagaagccagtgaagaagaatatttgaaatgaccaagtaggccttagctgatcttgaaataataatttcagtggactagtgaagcaaaaacctgtttggaaatgtaaagtgaaatgggttgaggatcagagacaattatcaagacaactatttcaagacatttggctattgaaggatagtcagaaaaggtggaaggtagttgtcatattgacagtttaatgcagtagtgtgggatcttttcaagatggcttgaaaatgtactaatgagaaaggagggagaactagaggtaacaaaatggttcctgagtcgtcagcttttaagtggtctttgggtaatgactgcaaagacatcaaatctggtgtattttcacaccacattcaacaatactgaaaaattacacgtggatcactttttaaaaaatctccactgtctattaatagtaaatgctcactaaatactttttgaggaaagataggaatgagagaaggaggagaaggaggagagaaagaaaaatgagaaaaggagccaaaaagaaatcccatattttatccttgttttcccttctactctcactacaattgtgcattctttctgatggaggttccccatttcataactcagtaacatataaaactttctggattgtctcatcattcgaaatgactgtgaacactctccaaaagagtgttctctttcttttattttttcctaactctcccctgttgttttcaatcagcctatggaaaaaaaaaaaaaatatatatatatatatataagccagctaggtaaaattttacacattttccaaagggtagccataagtgagttattcaatgtcaaatgaagacatcaaaacctgtctggacaatcagtggtaatgtcatttatatattttttcattgaaagtattccatacactgaaacctccacatatgaaatataaagtcttgaaatttataaattatagtacaaactattttcattatctttcatttgtcttatttattacaaacttgcctagtgcttgtgtaatataattcaaggtaaaaattactgttcaattttgtgaacttatttttttcccatgaaactcattctagatacaggcattttttcccccaaactgactcttctaaatgttgctttaattaaaatgaaatgaaggtttataaatttgcagtttgtgatatgttaaatccctgtttcaaattatatctcaagtattctgacatttatttctaaatcattactttgtctctgatcaaccataacttttacaatgcatttactgtttcatgtgaattatataagcagagtttcagtccccatgaactctcaactactgttgcacaaggattttggaaaaaaaaaaaaaagaaaaaagaaacagtaatgctcacctctccatagctcatttggggagaatattacctaaatttgttcctaatgcaagattgaaattaatcttgatttcccatcaaatgtacaaggattttacaatatagttcataatcgtgtttaatttctccagggtacaagttaagataaacaagtcactgacagtgtttatctataaatagagcagatggtctggggctgaggttagttatcaacttttctgactttaatttcatggttataaaacgctgtaaacctcactgtttataaaaggcagggaaggaactccagtgggcttcagtagccaagaaaccctcagtaacattaatctttctaactgatattcggtatcctcctagggtgcaatatttaagattgtggagtgattgctagacaaatttaaattttcactgggataattagctaacatttctgtcactgatctattataacgttgttaatgagttccatgtgagagaaatttagtaaatgagatgattctttctaaactctgctaggtgagtgtttaacaattaaggcagttacatatctaaaaaaagccttttttctttcaaaataatacttttttcttctgcaaagatgaactgtaatacccaactagactaaatgtacttagggatagaatttcataaggaaaaaccatagcatcatttaaataattaataatcatctaatgtatattgtatatacttaggccatgaatccagctacagcttttttttaaaaaaggccatagaacttaaaaagaagtaaaactattgattcttcatattctgaattgatttaaatacacaattttattgtgatcatttattttgctaaaggtctgtatgatcaatgtgattaaaattaatttttttcaaggaccccttattaaaaaaaagtattatttaaaatttctcatttttccccttgcaactttatagtgaatataaaagtaattttacaatcacaaaagtaaaaaataattcacaagttctacctctattacttttacattcttaagtggtttattttgcattctaacaagggggaagctttttttttttttttttctggagtcagagtcttggtgttttcacccaggctggagtgtagtggcttgatcacagctacgtcaatctggaatgcctgggctcaagtgatcctcacacctcagcctccagagaagtttggactacaggtgtgcaccaccatgcccagctaatctttaaactttttagagatggggtcttgctatgttggccaggctggcttcaaactcctgggctcaagtgatcttcccaacttagccttccaaagtgctggttttacaggcatcagccacattggaggtttcttaaatagatggtaatccaatatgcaaattggagactaaaactattttaaaaaaatgccggccgggcgcggtggctcacgcctgtaatcccagcactttgggaggccgaggcgggtggatcatgaggtcaggagatcgagaccatcctggctaacaaggtgaaaccccgtctctactaaaaatacaaaaaattagccgggcgcagtggcgggcgcctgtagtcccagctactcgggaggctgaggcaggagaatggcgtgaacccgggaagcggagcttgcagtgagccgagattgcgccactgcagtccgcagtccggcctgggcgacagagcgagactccgtctcaaaaaaaaaaaaaaaaaaaaaaaaaatgccttaactgtatttgagttcagactccctgagaatgagttttctaatgacaaaatcctcacttttctagtcttgtgttgggctgctgctttctgacccactctgggaggtttactactggtctgaaactccaatctatctctctactgattattgttaacacagtgctcaaatcttggctcccaataagctgtcttctgaatagcagcagccctaggtggagagataactgaatggaacatttgctaataaagtcatgtacctcgtaaggacattctggtcaatgacagacagacagactatacatcagtggtcccataagattataataccgtattttttatagtatcttttctatgtttatatgcttaaatatgcaaatatttaccattgcattaaagttgcctaaagtatttagtacaatagcacacactgtgcatgtttgtaacctaaaaacaaaggctatattatatagcctaggcatgtggtaggctataccacccaggttggtgtaagtacactctatgatgttcacacaagcacaaaatcgactaagcatgcatttttcagtgcatatccccatcattaagcaatgcatgactgtagattttcttatctcccttcctgctcagagtctgttgtcactagttttcatcggatgtaatatcccactgtttgatacattcatttttgtaaacaactgtctactcatagttagtgtcaggtctcaaaaatgcaggaagcatctataacagaagaccgcaacctctctaaaatgggagctttatctcatttttcttactgcctcaaaaccagctttcattacataaattggttactaaactattggtatgtttgacattcatatttgtgtacaattactcaaaactcggagtgatttcactttaaagttattgataaaaatcacctaaaagagatctatcagttaattgtaacaattgcatctttctgttgttaaagtagaaaagccagagaaaagattgtcctcacagggaaagatttgtttttatgaactggtcactctaaagcatgatttctaaaattgtgagctattggaaactggtgggaatgtatttctcagaaacatggccaagaagactagcacctcagaatggccaggaatagctctgaagggaggcaaaaataggtaacaggagaaactgaagttttagctaatagagagaaaaagagaacaagggaaaaaagcaaaactaggtattccagtatctgagtgcagaggtacattaaaataatcacttttgtaaagaaaggatctttttcaatatcccaaagatggcctaaagtaaccatcttttatttttcttgtctgtatataagatacaatgatttatgttataaaatataatcattgtactaatcttggtttgcaaaaaataaaagcttatacacggaaattacctgattaaaaggggaaaaacaggctgttaaaatttaagaaaattgttcctagttttattcaaatctatcagattaaaataatgtaatggaaataaattgctgccttaaaagataaagcaaattgtaatccataaaattaaaataatgtatgatatgtaactaatctcatttttatgattttctttcagattatccaaccctgtctaatgtcaaaggcatggcattgtatacaagaaaacatgcaaacaaaatcactttaactggatttcattcccccttcaatggtcagttaaaaatcaatcctctataatatttatattatttatttcctctaaaaatccagtgactattatttcttaatctttttctttttctaggagaagtaatctatgctgccatgtgcatgacagtcacctgtggaatccttctgttggttatggtcaagcttaggtaactgaatataaattagaaggaaaggtctgaaagggagtcacttagctgtgttaaagcatgttgcacaatggctgagcttacaaagagcctgagaatgaaagcttctctgttaagacatattaaatcaagttttatgtggcataggtccatggaaacgttactttcagtcttcctacataaggaaaatgtgatcataggagattttttatgttgcatttcataagcacatatgcattgtatgttccttccaattaaactcttatccatctttccccttggcttccctaccaaatccaaattgaactttgctgcatttgttattcaaatcatttgcatgattgataggctcacataactgacctattgtttactgcatacagtttgtatttacctgaagatgtattcttcactctaatatcttatatgctaatacattttattcatttttaataggcaattattgaaaaagacatttcataaagcctcacagagtgcccctagaaagacattaccattgcctgacattaatttattctccaaatcttggctgcttttattgctggaatgtagtaatgctccagcaggcatgtgagacattgagatgagatatacatcaacctctagatttctaaacgtctagtgtttaaaatttttccacttatttagcatttacaactatacataaaatagtgtagacttgcctttaattaaaaaaaactcacatttaaacatcaatcatgttcatttgcttattctttacacatatgggtacatgtctataaaatttgagtagcataaatgttaatgaagaaatatacataagtgtgtatacagccatatatacatgtaagtacatacacaaattatatcagtaagattgggccttcagaggaacagaagtattcactggagatttaccttatgacatctgacacctagaaagattaattcagtcaactctacaatacatataaacatatcttgctcctccagagatctcagacttaaaaaggccttgacaattaggcaaataaaagactggcatgagaaggtgtacggtgataccaaggggtcaggtacatacggacatcctaatttatttatttttaaatgcaatgccagctaaacaaaatgtatccactgtttggacccaatccctctaagcatttaatttgttgttaactaaaatcagtaccaaaacacactgcttttctccaaggccttaaaagttacatttgtatgagaagacattccgtgggttctaagatatgggttgaaagccaaataattagagtccattgctaagagggaaaaatagcatttggaatttattaaagtttactttatttggttttaagtacttgagaacactgtttagttattgttcctgcctagatattccatgacaaacattgttacaacaaaatatggacagttttctggcccggcaaaaacatcttactttaatggttctcaatctttacttcttaactacatacagaatgtataaaatttacacctgttccatgatcccactggtttttagatactactgttttgctacagatacaagatatagactactcataattccctatgtatttgctgtaacttcgtcttttttctcacctgcatagaaggcatatcccttttttggatggcagtgggggcattattattatggacaaatgttttgaatttattctaatgtgtattttaaagcaaattattcatactattaaatatatttgtatttagttacaaattattttcatataatttaaaatttatcataatgtgtaatcggaaaactccaggcccaggataaaagagacaaaatttaaagccatcataaaaagaacaaactgaaacaaaagcatcattggcaacaaaacctgtgttgccccacacctggagataaataatgctccctaaagaaagaagaatgattgctatttcagacattgttcactcacctgatggtcaagcccaacccatgtgaatacctgtcttctgtaaggaataagatagttgcatttgtttcatgttatgctatattcaaatagcccagagccttcaaagaagtttgcagagaaacaactaaaaatttaaatatttacaaaaagaaaggactttttaaaaaatgattacttggacatcatagttaaaggtgtgatgctccctagaaagaaaatatgatattttactattgggactttacattctggaacttgattagttttttcctccaggtgcagactccagcaaaaatgcaaacacacacaagcacatttgtgaaatccttaaaatggcatgttgttaacttttacttttattttatacagaacttccagaatatcaagtaaagcaagagatccttcatcgatccaaatacctggagaactctgattcattaggagtcatggacctataacaatcactcttttctctgcttttcttctttcctcttttcttctctcctctcctctcctctcttctcctctcctcccctcccctctctgtttctttttctttttcttttcttttttgtggcggagttttgctcttgttgcccaggctgcagtacaatggctcaatctcggttcactgcaacctctgcctccaaggttcaagtgattttcctgcctcagccttcccgagtagctgggattacaggtacccgccaccacgcccagctaatttttttgtatttttagtagagatggggttttgccaaattggccagggtggtctcaaactcctgacctcaggtgatccacccacctcggcctcccaaagtgctgggattacaggcgtgagcaaccacgtcaagacaacaatcactttctttaaagcaaatcctacagctggtcaacaccctattccatctgtcatcgagaaagaaaatgttaaaatagacttaaaaatattgctttgttacatataataatatggcatgatgatgttatttttttcttaatactcaagaaaaaatatatggtggtatcttttacaacactggaacagaaataaagtttcccttgaaggc

SEQ ID NO: 2 - RNA, 1911 nt, Homo sapiens
  source 1..1911: mol_type = mRNA
ttattctggacagttactcttaagaaagttgtcagaagaaacgcatctgcctttttttccaggtgaactgccgtgagttgtccagcatgatagtgtttattttcttggctatggggttaagcttggaaaatgaatacacttcccaaaccaataattgcacatatttaagagagcaatgcttacgtgatgcaaatggatgtaaacatgcttggagagtaatggaagatgcctgcaatgattcagatccaggtgacccctgcaagatgaggaattcatcatactgtaacctgagtatccagtacttagtggaaagcaatttccaatttaaagagtgtctttgcactgatgacttctattgtactgtgaacaaactgcttggaaaaaaatgtatcaataaatcagataacgtgaaagaggataaattcaaatggaatctaactacacgttcccatcatggattcaaagggatgtggtcctgtttggaagtggcagaggcatgtgtaggggatgtggtctgtaatgcacagttggcctcttaccttaaagcttgctcagcaaatggaaatccgtgtgatctgaaacagtgccaagcagccatacggttcttctatcaaaatataccttttaacattgcccagatgttggctttttgtgactgtgctcaatctgatataccttgtcagcagtccaaagaagctcttcacagcaagacatgtgcagtgaacatggttccaccccctacttgcctcagtgtaattcgcagctgccaaaatgatgaattatgcaggaggcactatagaacatttcagtcaaaatgctggcagcgtgtgactagaaagtgccatgaagatgagaattgcattagcaccttaagcaaacaggacctcacttgttcaggaagtgatgactgcaaagctgcttacatagatatccttgggacggtccttcaagtgcaatgtacctgtaggaccattacacaaagtgaggaatctttgtgtaagattttccagcacatgcttcatagaaaatcatgtttcaattatccaaccctgtctaatgtcaaaggcatggcattgtatacaagaaaacatgcaaacaaaatcactttaactggatttcattcccccttcaatggagaagtaatctatgctgccatgtgcatgacagtcacctgtggaatccttctgttggttatggtcaagcttagaacttccagaatatcaagtaaagcaagagatccttcatcgatccaaatacctggagaactctgattcattaggagtcatggacctataacaatcactcttttctctgcttttcttctttcctcttttcttctctcctctcctctcctctcttctcctctcctcccctcccctctctgtttctttttctttttcttttcttttttgtggcggagttttgctcttgttgcccaggctgcagtacaatggctcaatctcggttcactgcaacctctgcctccaaggttcaagtgattttcctgcctcagccttcccgagtagctgggattacaggtacccgccaccacgcccagctaatttttttgtatttttagtagagatggggttttgccaaattggccagggtggtctcaaactcctgacctcaggtgatccacccacctcggcctcccaaagtgctgggattacaggcgtgagcaaccacgtcaagacaacaatcactttctttaaagcaaatcctacagctggtcaacaccctattccatctgtcatcgagaaagaaaatgttaaaatagacttaaaaatattgctttgttacatataataatatggcatgatgatgttatttttttcttaatactcaagaaaaaatatatggtggtatcttttacaacactggaacagaaataaagtttcccttgaaggc

SEQ ID NO: 3 - DNA, 20 bp, synthetic construct
  source 1..20: mol_type = other DNA
tgtaggggatgtggtctgta

SEQ ID NO: 4 - DNA, 20 bp, synthetic construct
  source 1..20: mol_type = other DNA
tggtctgtaatgcacagttg

SEQ ID NO: 5 - DNA, 20 bp, synthetic construct
  source 1..20: mol_type = other DNA
gtctgtaatgcacagttggc

SEQ ID NO: 6 - DNA, 20 bp, synthetic construct
  source 1..20: mol_type = other DNA
cttaccttaaagcttgctca

SEQ ID NO: 7 - DNA, 19 bp, synthetic construct
  source 1..19: mol_type = other DNA
ggttcttctatcaaaatat

SEQ ID NO: 8 - DNA, 22 bp, synthetic construct
  source 1..22: mol_type = other DNA
ggttcttctatcaaaatatacc

SEQ ID NO: 9 - DNA, 22 bp, synthetic construct
  source 1..22: mol_type = other DNA
ttcttctatcaaaatatacctt

SEQ ID NO: 10 - DNA, 20 bp, synthetic construct
  source 1..20: mol_type = other DNA
cccagatgttggctttttgt

SEQ ID NO: 11 - DNA, 20 bp, synthetic construct
  source 1..20: mol_type = other DNA
ccagatgttggctttttgtg

SEQ ID NO: 12 - DNA, 20 bp, synthetic construct
  source 1..20: mol_type = other DNA
cagatgttggctttttgtga

SEQ ID NO: 13 - DNA, 20 bp, synthetic construct
  source 1..20: mol_type = other DNA
agatgttggctttttgtgac

SEQ ID NO: 14 - DNA, 20 bp, synthetic construct
  source 1..20: mol_type = other DNA
aaatgatgaattatgcagga

SEQ ID NO: 15 - DNA, 20 bp, synthetic construct
  source 1..20: mol_type = other DNA
gaaagtgccatgaagatgag

SEQ ID NO: 16 - DNA, 20 bp, synthetic construct
  source 1..20: mol_type = other DNA
aaagtgccatgaagatgaga

SEQ ID NO: 17 - DNA, 20 bp, synthetic construct
  source 1..20: mol_type = other DNA
attttccagcacatgcttca

SEQ ID NO: 18 - DNA, 20 bp, synthetic construct
  source 1..20: mol_type = other DNA
ttttccagcacatgcttcat

SEQ ID NO: 19 - DNA, 20 bp, synthetic construct
  source 1..20: mol_type = other DNA
tacagaccacatcccctaca

SEQ ID NO: 20 - DNA, 20 bp, synthetic construct
  source 1..20: mol_type = other DNA
caactgtgcattacagacca

SEQ ID NO: 21 - DNA, 20 bp, synthetic construct
  source 1..20: mol_type = other DNA
gccaactgtgcattacagac

SEQ ID NO: 22 - DNA, 20 bp, synthetic construct
  source 1..20: mol_type = other DNA
tgagcaagctttaaggtaag

SEQ ID NO: 23 - DNA, 19 bp, synthetic construct
  source 1..19: mol_type = other DNA
atattttgatagaagaacc

SEQ ID NO: 24 - DNA, 22 bp, synthetic construct
  source 1..22: mol_type = other DNA
ggtatattttgatagaagaacc

SEQ ID NO: 25 - DNA, 22 bp, synthetic construct
  source 1..22: mol_type = other DNA
aaggtatattttgatagaagaa

SEQ ID NO: 26 - DNA, 20 bp, synthetic construct
  source 1..20: mol_type = other DNA
acaaaaagccaacatctggg

SEQ ID NO: 27 - DNA, 20 bp, synthetic construct
  source 1..20: mol_type = other DNA
cacaaaaagccaacatctgg

SEQ ID NO: 28 - DNA, 20 bp, synthetic construct
  source 1..20: mol_type = other DNA
tcacaaaaagccaacatctg

SEQ ID NO: 29 - DNA, 20 bp, synthetic construct
  source 1..20: mol_type = other DNA
gtcacaaaaagccaacatct

SEQ ID NO: 30 - DNA, 20 bp, synthetic construct
  source 1..20: mol_type = other DNA
tcctgcataattcatcattt

SEQ ID NO: 31 - DNA, 20 bp, synthetic construct
  source 1..20: mol_type = other DNA
ctcatcttcatggcactttc

SEQ ID NO: 32 - DNA, 20 bp, synthetic construct
  source 1..20: mol_type = other DNA
tctcatcttcatggcacttt

SEQ ID NO: 33 - DNA, 20 bp, synthetic construct
  source 1..20: mol_type = other DNA
tgaagcatgtgctggaaaat

SEQ ID NO: 34 - DNA, 20 bp, synthetic construct
  source 1..20: mol_type = other DNA
atgaagcatgtgctggaaaa

SEQ ID NO: 35 - DNA, 23 bp, synthetic construct
  source 1..23: mol_type = other DNA
ggtgtgaaccatgagaagtatga

SEQ ID NO: 36 - DNA, 22 bp, synthetic construct
  source 1..22: mol_type = other DNA
gagtccttccacgataccaaag

SEQ ID NO: 37 - DNA, 24 bp, synthetic construct
  source 1..24: mol_type = other DNA
agatcatcagcaatgcctcctgca